European Patent Application EP 4 368 209 A1, published May 15, 2024. Title: CARDIAC VASCULAR ENDOTHELIAL CELL-DERIVED NUCLEIC ACID REGULATORY ELEMENTS AND METHODS AND USE THEREOF. Applicant: Vrije Universiteit Brussel. The sequence listing filed with the application follows.

SEQUENCE LISTING (22 sequences)

SEQ ID NO: 1 - DNA, 426 bp, Homo sapiens
  source 1..426: mol_type = genomic DNA; note = CV-EC-CRE3
ccctaaggagaggaaaagtgggggagggaaggggactctggaggagcaaaagcaagaggcctgggggcgactggggtggggcgtctcctagagcgaggattgctgcagagtgcgcgtgcacgcccgcacatccacacccacggctacacatcatatctgcacacgcacaaaaccacacaccctcccacgccggtcccatatcctttctgcggggtgagcagcagattcccggaaagggggaaatgtagccgcaaaagcaaagccgggggcctggcgcccactctggcggcgactacagcccccacgctgggcacactgcgagctgggggtgcccggcgcgggagaagccgcgcccagccgggctggtagcccagcggggggcgcggcagggcgaggagcagcccgcgctgctcccgcccctcgggt

SEQ ID NO: 2 - DNA, 522 bp, Homo sapiens
  source 1..522: mol_type = genomic DNA; note = CV-EC-CRE9
aggcgggaggtcagggggcgatgggtggtgggaaggccagtgtccacccagggcccaccagtgggtgggggacagagggacagtcatggaaaatctgagtgtgatctacagtcacgaaccacctgctcagggacagatggagacatctttcccagtagctggaatcagaactttcccctgaaatccacagcccggtaactcactctcttatctctgaccctccggaagccagagatctagctatttcatcagcatggacttttctttctgtgcccgtgtgaccccttacaaaagagctcaagctggaaagagaggattggatcaagaaagagagaacttaggattcaggggaaaaggggaaagtgataaccccttgagtcagattctgagaagagggtttctctgagaggtcggtggggagcagcccgcaggcagctggaccctggtatggaagggctcggctcctaaggcaggtaagagaaggcagggccacgtgcatgaagtagaggcaggggtcatggc

SEQ ID NO: 3 - DNA, 408 bp, Homo sapiens
  source 1..408: mol_type = genomic DNA; note = CV-EC-CRE18
tccgggttttccccattcccagctcggctgcaaccgagagacagacggaagaaactgccaatggaaggacgcaaagcgtcaactttgtgttcgcccgccactctcggccaatgtgcgctcgtgtctccggagtcccgccttccgtgtcgggcgcccccttttggcagcacagggacgaaccctacgtctcgccatcttgtgtgtggcacaggtaaatttctggactatctttccacctattctggtcctttttcccacacaaccgatttcttagttcgacagctaagtgcggtggcgataaggccagcgtagcctgttgttctcggatcgcccacgtgagctagatcgctacgtcacgccacgcttgccgagcccggcgccatcttgagtgtggcgttttgatgctcc

SEQ ID NO: 4 - DNA, 5753 bp, synthetic construct
  source 1..5753: mol_type = other DNA; note = AAVss- IFI27-EC-CRE1b-ICAM2-Luc-pA
acatgtcctgcaggcagctgcgcgctcgctcgctcactgaggccgcccgggcaaagcccgggcggcctcagtgagcgagcgagcgcgcagagagggagtggccaactccatcactaggggttcctgcggccggcgcgccacgcgtggtaccgagactttttttgaaaaacggaacatctgcctatcgcaaggactactattattctgaaaatcaccttcttcattagaaagtaatatttatcattttattatagaactttgatcttacttcttgtgacttcattctgcgtagagcacactcccatccttgaattaaatgacaaagcattttatattaactgacaatgactgatgccatgggcaaatcctatttctgtaaataactgaattttcttctggactgcgcatgaggggagaaagatgtctgcagtttcggtttcctggaaaatgaaacctatctcatttgttgcctgtgtcaaggggcagtgcttcagtcggggtggagctgcttaaaaggcctgggatcacaccctttgggaacacatccaagcttaagacggtgaggtcagcttcacattctcaggaactctccttctttgggtaagactgggagggtgggcaggagctacccttcccgtggccccggaccttgggtgggctgtgggctcagggagcggaggggaggccttaagcatccactctctgcccggtgtttttgttccgtacgcggtctagaattcctgcagggcccactagtctcccaggcatgactccaacaatgcatcccatgggatttggggttccccagatctggggcttgtaggcctgactctcccctgtgcacacgtctcatacacgcatgcgtgcacccattgcctgccccgccccttgcacagggagtcagcagggaggactgggttatgccctgcttatcagcagcttcccagcttcctctgcctggattcttagaggcctggggtcctagaacgagctggtgcacgtggcttcccaaagatctctcagataatgagaggaaatgcagtcatcagtttgcagaaggctagggattctgggccatagctcagacctgcgcccaccatctccctccaggcagcccttggctggtccctgcgagcccgtggagactgccagtcgctagaaagaggtaagggtttaagggatggttggttggtggggtattaatgtttaattacctggagcacctgcctgaaatcactttttttcaggttggaagcttatggaagatgccaaaaacattaagaagggcccagcgccattctacccactcgaagacgggaccgccggcgagcagctgcacaaagccatgaagcgctacgccctggtgcccggcaccatcgcctttaccgacgcacatatcgaggtggacattacctacgccgagtacttcgagatgagcgttcggctggcagaagctatgaagcgctatgggctgaatacaaaccatcggatcgtggtgtgcagcgagaatagcttgcagttcttcatgcccgtgttgggtgccctgttcatcggtgtggctgtggccccagctaacgacatctacaacgagcgcgagctgctgaacagcatgggcatcagccagcccaccgtcgtattcgtgagcaagaaagggctgcaaaagatcctcaacgtgcaaaagaagctaccgatcatacaaaagatcatcatcatggatagcaagaccgactaccagggcttccaaagcatgtacaccttcgtgacttcccatttgccacccggcttcaacgagtacgacttcgtgcccgagagcttcgaccgggacaaaaccatcgccctgatcatgaacagtagtggcagtaccggattgcccaagggcgtagccctaccgcaccgcaccgcttgtgtccgattcagtcatgcccgcgaccccatcttcggcaaccagatcatccccgacaccgctatcctcagcgtggtgccatttcaccacggcttcggcatgttcaccacgctgggctacttgatctgcggctttcgggtcgtgctcatgtaccgcttcgaggaggagctattcttgcgcagcttgcaagactataagattcaatctgccctgctggtgcccacactatttagcttcttcgctaagagcactctcatcgacaagtacgacctaagcaacttgcacgagatcgccagcggcggggcgccgctcagcaaggaggtaggtgaggccgtggccaaacgcttccacctaccaggcatccgccagggctacggcctgacagaaacaaccagcgccattctgatcacccccgaaggggacgacaagcctggcgcagtaggcaaggtggtgcccttcttcgaggctaaggtggtggacttggacaccggtaagacactgggtgtgaaccagcgcggcgagctgtgcgtccgtggccccatgatcatgagcggctacgttaacaaccccgaggctacaaacgctctcatcgacaaggacggctggctgcacagcggcgacatcgcctactgggacgaggacgagcacttcttcatcgtggaccggctgaagagcctgatcaaatacaagggctaccaggtagccccagccgaactggagagcatcctgctgcaacaccccaacatcttcgacgccggggtcgccggcctgcccgacgacgatgccggcgagctgcccgccgcagtcgtcgtgctggaacacggtaaaaccatgaccgagaaggagatcgtggactatgtggccagccaggttacaaccgccaagaagctgcgcggtggtgttgtgttcgtggacgaggtgcctaaaggactgaccggcaagttggacgcccgcaagatccgcgagattctcattaaggccaagaagggcggcaagatcgccgtgtaattcgaaacgttgagtccatcttgagcatctgacttctggctaaataaaagatctttattttcattagatctgtgtgttggttttttgtgtgcgtcgagatccacggccgcaggaacccctagtgatggagttggccactccctctctgcgcgctcgctcgctcactgaggccgggcgaccaaaggtcgcccgacgcccgggctttgcccgggcggcctcagtgagcgagcgagcgcgcagctgcctgcaggggcgcctgatgcggtattttctccttacgcatctgtgcggtatttcacaccgcatacgtcaaagcaaccatagtacgcgccctgtagcggcgcattaagcgcggcgggtgtggtggttacgcgcagcgtgaccgctacacttgccagcgccctagcgcccgctcctttcgctttcttcccttcctttctcgccacgttcgccggctttccccgtcaagctctaaatcgggggctccctttagggttccgatttagtgctttacggcacctcgaccccaaaaaacttgatttgggtgatggttcacgtagtgggccatcgccctgatagacggtttttcgccctttgacgttggagtccacgttctttaatagtggactcttgttccaaactggaacaacactcaaccctatctcgggctattcttttgatttataagggattttgccgatttcggcctattggttaaaaaatgagctgatttaacaaaaatttaacgcgaattttaacaaaatattaacgtttacaattttatggtgcactctcagtacaatctgctctgatgccgcatagttaagccagccccgacacccgccaacacccgctgacgcgccctgacgggcttgtctgctcccggcatccgcttacagacaagctgtgaccgtctccgggagctgcatgtgtcagaggttttcaccgtcatcaccgaaacgcgcgagacgaaagggcctcgtgatacgcctatttttataggttaatgtcatgataataatggtttcttagacgtcaggtggcacttttcggggaaatgtgcgcggaacccctatttgtttatttttctaaatacattcaaatatgtatccgctcatgagacaataaccctgataaatgcttcaataatattgaaaaaggaagagtatgagtattcaacatttccgtgtcgcccttattcccttttttgcggcattttgccttcctgtttttgctcacccagaaacgctggtgaaagtaaaagatgctgaagatcagttgggtgcacgagtgggttacatcgaactggatctcaacagcggtaagatccttgagagttttcgccccgaagaacgttttccaatgatgagcacttttaaagttctgctatgtggcgcggtattatcccgtattgacgccgggcaagagcaactcggtcgccgcatacactattctcagaatgacttggttgagtactcaccagtcacagaaaagcatcttacggatggcatgacagtaagagaattatgcagtgctgccataaccatgagtgataacactgcggccaacttacttctgacaacgatcggaggaccgaaggagctaaccgcttttttgcacaacatgggggatcatgtaactcgccttgatcgttgggaaccggagctgaatgaagccataccaaacgacgagcgtgacaccacgatgcctgtagcaatggcaacaacgttgcgcaaactattaactggcgaactacttactctagcttcccggcaacaattaatagactggatggaggcggataaagttgcaggaccacttctgcgctcggcccttccggctggctggtttattgctgataaatctggagccggtgagcgtgggtctcgcggtatcattgcagcactggggccagatggtaagccctcccgtatcgtagttatctacacgacggggagtcaggcaactatggatgaacgaaatagacagatcgctgagataggtgcctcactgattaagcattggtaactgtcagaccaagtttactcatatatactttagattgatttaaaacttcatttttaatttaaaaggatctaggtgaagatcctttttgataatctcatgaccaaaatcccttaacgtgagttttcgttccactgagcgtcagaccccgtagaaaagatcaaaggatcttcttgagatcctttttttctgcgcgtaatctgctgcttgcaaacaaaaaaaccaccgctaccagcggtggtttgtttgccggatcaagagctaccaactctttttccgaaggtaactggcttcagcagagcgcagataccaaatactgtccttctagtgtagccgtagttaggccaccacttcaagaactctgtagcaccgcctacatacctcgctctgctaatcctgttaccagtggctgctgccagtggcgataagtcgtgtcttaccgggttggactcaagacgatagttaccggataaggcgcagcggtcgggctgaacggggggttcgtgcacacagcccagcttggagcgaacgacctacaccgaactgagatacctacagcgtgagctatgagaaagcgccacgcttcccgaagggagaaaggcggacaggtatccggtaagcggcagggtcggaacaggagagcgcacgagggagcttccagggggaaacgcctggtatctttatagtcctgtcgggtttcgccacctctgacttgagcgtcgatttttgtgatgctcgtcaggggggcggagcctatggaaaaacgccagcaacgcggcctttttacggttcctggccttttgctggccttttgctc

SEQ ID NO: 5 - DNA, 6173 bp, synthetic construct
  source 1..6173: mol_type = other DNA; note = AAVss-CV-EC-CRE3- IFI27-EC-CRE1b-ICAM2-Luc-pA
acatgtcctgcaggcagctgcgcgctcgctcgctcactgaggccgcccgggcaaagcccgggcggcctcagtgagcgagcgagcgcgcagagagggagtggccaactccatcactaggggttcctgcggccggcgcgccccctaaggagaggaaaagtgggggagggaaggggactctggaggagcaaaagcaagaggcctgggggcgactggggtggggcgtctcctagagcgaggattgctgcagagtgcgcgtgcacgcccgcacatccacacccacggctacacatcatatctgcacacgcacaaaaccacacaccctcccacgccggtcccatatcctttctgcggggtgagcagcagattcccggaaagggggaaatgtagccgcaaaagcaaagccgggggcctggcgcccactctggcggcgactacagcccccacgctgggcacactgcgagctgggggtgcccggcgcgggagaagccgcgcccagccgggctggtagcccagcggggggcgcggcagggcgaggagcagcccgcgctgctcccgcccctcgggtggtaccgagactttttttgaaaaacggaacatctgcctatcgcaaggactactattattctgaaaatcaccttcttcattagaaagtaatatttatcattttattatagaactttgatcttacttcttgtgacttcattctgcgtagagcacactcccatccttgaattaaatgacaaagcattttatattaactgacaatgactgatgccatgggcaaatcctatttctgtaaataactgaattttcttctggactgcgcatgaggggagaaagatgtctgcagtttcggtttcctggaaaatgaaacctatctcatttgttgcctgtgtcaaggggcagtgcttcagtcggggtggagctgcttaaaaggcctgggatcacaccctttgggaacacatccaagcttaagacggtgaggtcagcttcacattctcaggaactctccttctttgggtaagactgggagggtgggcaggagctacccttcccgtggccccggaccttgggtgggctgtgggctcagggagcggaggggaggccttaagcatccactctctgcccggtgtttttgttccgtacgcggtctagaattcctgcagggcccactagtctcccaggcatgactccaacaatgcatcccatgggatttggggttccccagatctggggcttgtaggcctgactctcccctgtgcacacgtctcatacacgcatgcgtgcacccattgcctgccccgccccttgcacagggagtcagcagggaggactgggttatgccctgcttatcagcagcttcccagcttcctctgcctggattcttagaggcctggggtcctagaacgagctggtgcacgtggcttcccaaagatctctcagataatgagaggaaatgcagtcatcagtttgcagaaggctagggattctgggccatagctcagacctgcgcccaccatctccctccaggcagcccttggctggtccctgcgagcccgtggagactgccagtcgctagaaagaggtaagggtttaagggatggttggttggtggggtattaatgtttaattacctggagcacctgcctgaaatcactttttttcaggttggaagcttatggaagatgccaaaaacattaagaagggcccagcgccattctacccactcgaagacgggaccgccggcgagcagctgcacaaagccatgaagcgctacgccctggtgcccggcaccatcgcctttaccgacgcacatatcgaggtggacattacctacgccgagtacttcgagatgagcgttcggctggcagaagctatgaagcgctatgggctgaatacaaaccatcggatcgtggtgtgcagcgagaatagcttgcagttcttcatgcccgtgttgggtgccctgttcatcggtgtggctgtggccccagctaacgacatctacaacgagcgcgagctgctgaacagcatgggcatcagccagcccaccgtcgtattcgtgagcaagaaagggctgcaaaagatcctcaacgtgcaaaagaagctaccgatcatacaaaagatcatcatcatggatagcaagaccgactaccagggcttccaaagcatgtacaccttcgtgacttcccatttgccacccggcttcaacgagtacgacttcgtgcccgagagcttcgaccgggacaaaaccatcgccctgatcatgaacagtagtggcagtaccggattgcccaagggcgtagccctaccgcaccgcaccgcttgtgtccgattcagtcatgcccgcgaccccatcttcggcaaccagatcatccccgacaccgctatcctcagcgtggtgccatttcaccacggcttcggcatgttcaccacgctgggctacttgatctgcggctttcgggtcgtgctcatgtaccgcttcgaggaggagctattcttgcgcagcttgcaagactataagattcaatctgccctgctggtgcccacactatttagcttcttcgctaagagcactctcatcgacaagtacgacctaagcaacttgcacgagatcgccagcggcggggcgccgctcagcaaggaggtaggtgaggccgtggccaaacgcttccacctaccaggcatccgccagggctacggcctgacagaaacaaccagcgccattctgatcacccccgaaggggacgacaagcctggcgcagtaggcaaggtggtgcccttcttcgaggctaaggtggtggacttggacaccggtaagacactgggtgtgaaccagcgcggcgagctgtgcgtccgtggccccatgatcatgagcggctacgttaacaaccccgaggctacaaacgctctcatcgacaaggacggctggctgcacagcggcgacatcgcctactgggacgaggacgagcacttcttcatcgtggaccggctgaagagcctgatcaaatacaagggctaccaggtagccccagccgaactggagagcatcctgctgcaacaccccaacatcttcgacgccggggtcgccggcctgcccgacgacgatgccggcgagctgcccgccgcagtcgtcgtgctggaacacggtaaaaccatgaccgagaaggagatcgtggactatgtggccagccaggttacaaccgccaagaagctgcgcggtggtgttgtgttcgtggacgaggtgcctaaaggactgaccggcaagttggacgcccgcaagatccgcgagattctcattaaggccaagaagggcggcaagatcgccgtgtaattcgaaacgttgagtccatcttgagcatctgacttctggctaaataaaagatctttattttcattagatctgtgtgttggttttttgtgtgcgtcgagatccacggccgcaggaacccctagtgatggagttggccactccctctctgcgcgctcgctcgctcactgaggccgggcgaccaaaggtcgcccgacgcccgggctttgcccgggcggcctcagtgagcgagcgagcgcgcagctgcctgcaggggcgcctgatgcggtattttctccttacgcatctgtgcggtatttcacaccgcatacgtcaaagcaaccatagtacgcgccctgtagcggcgcattaagcgcggcgggtgtggtggttacgcgcagcgtgaccgctacacttgccagcgccctagcgcccgctcctttcgctttcttcccttcctttctcgccacgttcgccggctttccccgtcaagctctaaatcgggggctccctttagggttccgatttagtgctttacggcacctcgaccccaaaaaacttgatttgggtgatggttcacgtagtgggccatcgccctgatagacggtttttcgccctttgacgttggagtccacgttctttaatagtggactcttgttccaaactggaacaacactcaaccctatctcgggctattcttttgatttataagggattttgccgatttcggcctattggttaaaaaatgagctgatttaacaaaaatttaacgcgaattttaacaaaatattaacgtttacaattttatggtgcactctcagtacaatctgctctgatgccgcatagttaagccagccccgacacccgccaacacccgctgacgcgccctgacgggcttgtctgctcccggcatccgcttacagacaagctgtgaccgtctccgggagctgcatgtgtcagaggttttcaccgtcatcaccgaaacgcgcgagacgaaagggcctcgtgatacgcctatttttataggttaatgtcatgataataatggtttcttagacgtcaggtggcacttttcggggaaatgtgcgcggaacccctatttgtttatttttctaaatacattcaaatatgtatccgctcatgagacaataaccctgataaatgcttcaataatattgaaaaaggaagagtatgagtattcaacatttccgtgtcgcccttattcccttttttgcggcattttgccttcctgtttttgctcacccagaaacgctggtgaaagtaaaagatgctgaagatcagttgggtgcacgagtgggttacatcgaactggatctcaacagcggtaagatccttgagagttttcgccccgaagaacgttttccaatgatgagcacttttaaagttctgctatgtggcgcggtattatcccgtattgacgccgggcaagagcaactcggtcgccgcatacactattctcagaatgacttggttgagtactcaccagtcacagaaaagcatcttacggatggcatgacagtaagagaattatgcagtgctgccataaccatgagtgataacactgcggccaacttacttctgacaacgatcggaggaccgaaggagctaaccgcttttttgcacaacatgggggatcatgtaactcgccttgatcgttgggaaccggagctgaatgaagccataccaaacgacgagcgtgacaccacgatgcctgtagcaatggcaacaacgttgcgcaaactattaactggcgaactacttactctagcttcccggcaacaattaatagactggatggaggcggataaagttgcaggaccacttctgcgctcggcccttccggctggctggtttattgctgataaatctggagccggtgagcgtgggtctcgcggtatcattgcagcactggggccagatggtaagccctcccgtatcgtagttatctacacgacggggagtcaggcaactatggatgaacgaaatagacagatcgctgagataggtgcctcactgattaagcattggtaactgtcagaccaagtttactcatatatactttagattgatttaaaacttcatttttaatttaaaaggatctaggtgaagatcctttttgataatctcatgaccaaaatcccttaacgtgagttttcgttccactgagcgtcagaccccgtagaaaagatcaaaggatcttcttgagatcctttttttctgcgcgtaatctgctgcttgcaaacaaaaaaaccaccgctaccagcggtggtttgtttgccggatcaagagctaccaactctttttccgaaggtaactggcttcagcagagcgcagataccaaatactgtccttctagtgtagccgtagttaggccaccacttcaagaactctgtagcaccgcctacatacctcgctctgctaatcctgttaccagtggctgctgccagtggcgataagtcgtgtcttaccgggttggactcaagacgatagttaccggataaggcgcagcggtcgggctgaacggggggttcgtgcacacagcccagcttggagcgaacgacctacaccgaactgagatacctacagcgtgagctatgagaaagcgccacgcttcccgaagggagaaaggcggacaggtatccggtaagcggcagggtcggaacaggagagcgcacgagggagcttccagggggaaacgcctggtatctttatagtcctgtcgggtttcgccacctctgacttgagcgtcgatttttgtgatgctcgtcaggggggcggagcctatggaaaaacgccagcaacgcggcctttttacggttcctggccttttgctggccttttgctc

SEQ ID NO: 6 - DNA, 6269 bp, synthetic construct
  source 1..6269: mol_type = other DNA; note = AAVss-CV-EC-CRE9- IFI27-EC-CRE1b-ICAM2-Luc-pA
acatgtcctgcaggcagctgcgcgctcgctcgctcactgaggccgcccgggcaaagcccgggcggcctcagtgagcgagcgagcgcgcagagagggagtggccaactccatcactaggggttcctgcggccggcgcgccaggcgggaggtcagggggcgatgggtggtgggaaggccagtgtccacccagggcccaccagtgggtgggggacagagggacagtcatggaaaatctgagtgtgatctacagtcacgaaccacctgctcagggacagatggagacatctttcccagtagctggaatcagaactttcccctgaaatccacagcccggtaactcactctcttatctctgaccctccggaagccagagatctagctatttcatcagcatggacttttctttctgtgcccgtgtgaccccttacaaaagagctcaagctggaaagagaggattggatcaagaaagagagaacttaggattcaggggaaaaggggaaagtgataaccccttgagtcagattctgagaagagggtttctctgagaggtcggtggggagcagcccgcaggcagctggaccctggtatggaagggctcggctcctaaggcaggtaagagaaggcagggccacgtgcatgaagtagaggcaggggtcatggcggtaccgagactttttttgaaaaacggaacatctgcctatcgcaaggactactattattctgaaaatcaccttcttcattagaaagtaatatttatcattttattatagaactttgatcttacttcttgtgacttcattctgcgtagagcacactcccatccttgaattaaatgacaaagcattttatattaactgacaatgactgatgccatgggcaaatcctatttctgtaaataactgaattttcttctggactgcgcatgaggggagaaagatgtctgcagtttcggtttcctggaaaatgaaacctatctcatttgttgcctgtgtcaaggggcagtgcttcagtcggggtggagctgcttaaaaggcctgggatcacaccctttgggaacacatccaagcttaagacggtgaggtcagcttcacattctcaggaactctccttctttgggtaagactgggagggtgggcaggagctacccttcccgtggccccggaccttgggtgggctgtgggctcagggagcggaggggaggccttaagcatccactctctgcccggtgtttttgttccgtacgcggtctagaattcctgcagggcccactagtctcccaggcatgactccaacaatgcatcccatgggatttggggttccccagatctggggcttgtaggcctgactctcccctgtgcacacgtctcatacacgcatgcgtgcacccattgcctgccccgccccttgcacagggagtcagcagggaggactgggttatgccctgcttatcagcagcttcccagcttcctctgcctggattcttagaggcctggggtcctagaacgagctggtgcacgtggcttcccaaagatctctcagataatgagaggaaatgcagtcatcagtttgcagaaggctagggattctgggccatagctcagacctgcgcccaccatctccctccaggcagcccttggctggtccctgcgagcccgtggagactgccagtcgctagaaagaggtaagggtttaagggatggttggttggtggggtattaatgtttaattacctggagcacctgcctgaaatcactttttttcaggttggaagcttatggaagatgccaaaaacattaagaagggcccagcgccattctacccactcgaagacgggaccgccggcgagcagctgcacaaagccatgaagcgctacgccctggtgcccggcaccatcgcctttaccgacgcacatatcgaggtggacattacctacgccgagtacttcgagatgagcgttcggctggcagaagctatgaagcgctatgggctgaatacaaaccatcggatcgtggtgtgcagcgagaatagcttgcagttcttcatgcccgtgttgggtgccctgttcatcggtgtggctgtggccccagctaacgacatctacaacgagcgcgagctgctgaacagcatgggcatcagccagcccaccgtcgtattcgtgagcaagaaagggctgcaaaagatcctcaacgtgcaaaagaagctaccgatcatacaaaagatcatcatcatggatagcaagaccgactaccagggcttccaaagcatgtacaccttcgtgacttcccatttgccacccggcttcaacgagtacgacttcgtgcccgagagcttcgaccgggacaaaaccatcgccctgatcatgaacagtagtggcagtaccggattgcccaagggcgtagccctaccgcaccgcaccgcttgtgtccgattcagtcatgcccgcgaccccatcttcggcaaccagatcatccccgacaccgctatcctcagcgtggtgccatttcaccacggcttcggcatgttcaccacgctgggctacttgatctgcggctttcgggtcgtgctcatgtaccgcttcgaggaggagctattcttgcgcagcttgcaagactataagattcaatctgccctgctggtgcccacactatttagcttcttcgctaagagcactctcatcgacaagtacgacctaagcaacttgcacgagatcgccagcggcggggcgccgctcagcaaggaggtaggtgaggccgtggccaaacgcttccacctaccaggcatccgccagggctacggcctgacagaaacaaccagcgccattctgatcacccccgaaggggacgacaagcctggcgcagtaggcaaggtggtgcccttcttcgaggctaaggtggtggacttggacaccggtaagacactgggtgtgaaccagcgcggcgagctgtgcgtccgtggccccatgatcatgagcggctacgttaacaaccccgaggctacaaacgctctcatcgacaaggacggctggctgcacagcggcgacatcgcctactgggacgaggacgagcacttcttcatcgtggaccggctgaagagcctgatcaaatacaagggctaccaggtagccccagccgaactggagagcatcctgctgcaacaccccaacatcttcgacgccggggtcgccggcctgcccgacgacgatgccggcgagctgcccgccgcagtcgtcgtgctggaacacggtaaaaccatgaccgagaaggagatcgtggactatgtggccagccaggttacaaccgccaagaagctgcgcggtggtgttgtgttcgtggacgaggtgcctaaaggactgaccggcaagttggacgcccgcaagatccgcgagattctcattaaggccaagaagggcggcaagatcgccgtgtaattcgaaacgttgagtccatcttgagcatctgacttctggctaaataaaagatctttattttcattagatctgtgtgttggttttttgtgtgcgtcgagatccacggccgcaggaacccctagtgatggagttggccactccctctctgcgcgctcgctcgctcactgaggccgggcgaccaaaggtcgcccgacgcccgggctttgcccgggcggcctcagtgagcgagcgagcgcgcagctgcctgcaggggcgcctgatgcggtattttctccttacgcatctgtgcggtatttcacaccgcatacgtcaaagcaaccatagtacgcgccctgtagcggcgcattaagcgcggcgggtgtggtggttacgcgcagcgtgaccgctacacttgccagcgccctagcgcccgctcctttcgctttcttcccttcctttctcgccacgttcgccggctttccccgtcaagctctaaatcgggggctccctttagggttccgatttagtgctttacggcacctcgaccccaaaaaacttgatttgggtgatggttcacgtagtgggccatcgccctgatagacggtttttcgccctttgacgttggagtccacgttctttaatagtggactcttgttccaaactggaacaacactcaaccctatctcgggctattcttttgatttataagggattttgccgatttcggcctattggttaaaaaatgagctgatttaacaaaaatttaacgcgaattttaacaaaatattaacgtttacaattttatggtgcactctcagtacaatctgctctgatgccgcatagttaagccagccccgacacccgccaacacccgctgacgcgccctgacgggcttgtctgctcccggcatccgcttacagacaagctgtgaccgtctccgggagctgcatgtgtcagaggttttcaccgtcatcaccgaaacgcgcgagacgaaagggcctcgtgatacgcctatttttataggttaatgtcatgataataatggtttcttagacgtcaggtggcacttttcggggaaatgtgcgcggaacccctatttgtttatttttctaaatacattcaaatatgtatccgctcatgagacaataaccctgataaatgcttcaataatattgaaaaaggaagagtatgagtattcaacatttccgtgtcgcccttattcccttttttgcggcattttgccttcctgtttttgctcacccagaaacgctggtgaaagtaaaagatgctgaagatcagttgggtgcacgagtgggttacatcgaactggatctcaacagcggtaagatccttgagagttttcgccccgaagaacgttttccaatgatgagcacttttaaagttctgctatgtggcgcggtattatcccgtattgacgccgggcaagagcaactcggtcgccgcatacactattctcagaatgacttggttgagtactcaccagtcacagaaaagcatcttacggatggcatgacagtaagagaattatgcagtgctgccataaccatgagtgataacactgcggccaacttacttctgacaacgatcggaggaccgaaggagctaaccgcttttttgcacaacatgggggatcatgtaactcgccttgatcgttgggaaccggagctgaatgaagccataccaaacgacgagcgtgacaccacgatgcctgtagcaatggcaacaacgttgcgcaaactattaactggcgaactacttactctagcttcccggcaacaattaatagactggatggaggcggataaagttgcaggaccacttctgcgctcggcccttccggctggctggtttattgctgataaatctggagccggtgagcgtgggtctcgcggtatcattgcagcactggggccagatggtaagccctcccgtatcgtagttatctacacgacggggagtcaggcaactatggatgaacgaaatagacagatcgctgagataggtgcctcactgattaagcattggtaactgtcagaccaagtttactcatatatactttagattgatttaaaacttcatttttaatttaaaaggatctaggtgaagatcctttttgataatctcatgaccaaaatcccttaacgtgagttttcgttccactgagcgtcagaccccgtagaaaagatcaaaggatcttcttgagatcctttttttctgcgcgtaatctgctgcttgcaaacaaaaaaaccaccgctaccagcggtggtttgtttgccggatcaagagctaccaactctttttccgaaggtaactggcttcagcagagcgcagataccaaatactgtccttctagtgtagccgtagttaggccaccacttcaagaactctgtagcaccgcctacatacctcgctctgctaatcctgttaccagtggctgctgccagtggcgataagtcgtgtcttaccgggttggactcaagacgatagttaccggataaggcgcagcggtcgggctgaacggggggttcgtgcacacagcccagcttggagcgaacgacctacaccgaactgagatacctacagcgtgagctatgagaaagcgccacgcttcccgaagggagaaaggcggacaggtatccggtaagcggcagggtcggaacaggagagcgcacgagggagcttccagggggaaacgcctggtatctttatagtcctgtcgggtttcgccacctctgacttgagcgtcgatttttgtgatgctcgtcaggggggcggagcctatggaaaaacgccagcaacgcggcctttttacggttcctggccttttgctggccttttgctc

SEQ ID NO: 7 - DNA, 6155 bp, synthetic construct
  source 1..6155: mol_type = other DNA; note = AAVss-CV-EC-CRE18- IFI27-EC-CRE1b-ICAM2-Luc-pA
acatgtcctgcaggcagctgcgcgctcgctcgctcactgaggccgcccgggcaaagcccgggcggcctcagtgagcgagcgagcgcgcagagagggagtggccaactccatcactaggggttcctgcggccggcgcgcctccgggttttccccattcccagctcggctgcaaccgagagacagacggaagaaactgccaatggaaggacgcaaagcgtcaactttgtgttcgcccgccactctcggccaatgtgcgctcgtgtctccggagtcccgccttccgtgtcgggcgcccccttttggcagcacagggacgaaccctacgtctcgccatcttgtgtgtggcacaggtaaatttctggactatctttccacctattctggtcctttttcccacacaaccgatttcttagttcgacagctaagtgcggtggcgataaggccagcgtagcctgttgttctcggatcgcccacgtgagctagatcgctacgtcacgccacgcttgccgagcccggcgccatcttgagtgtggcgttttgatgctccggtaccgagactttttttgaaaaacggaacatctgcctatcgcaaggactactattattctgaaaatcaccttcttcattagaaagtaatatttatcattttattatagaactttgatcttacttcttgtgacttcattctgcgtagagcacactcccatccttgaattaaatgacaaagcattttatattaactgacaatgactgatgccatgggcaaatcctatttctgtaaataactgaattttcttctggactgcgcatgaggggagaaagatgtctgcagtttcggtttcctggaaaatgaaacctatctcatttgttgcctgtgtcaaggggcagtgcttcagtcggggtggagctgcttaaaaggcctgggatcacaccctttgggaacacatccaagcttaagacggtgaggtcagcttcacattctcaggaactctccttctttgggtaagactgggagggtgggcaggagctacccttcccgtggccccggaccttgggtgggctgtgggctcagggagcggaggggaggccttaagcatccactctctgcccggtgtttttgttccgtacgcggtctagaattcctgcagggcccactagtctcccaggcatgactccaacaatgcatcccatgggatttggggttccccagatctggggcttgtaggcctgactctcccctgtgcacacgtctcatacacgcatgcgtgcacccattgcctgccccgccccttgcacagggagtcagcagggaggactgggttatgccctgcttatcagcagcttcccagcttcctctgcctggattcttagaggcctggggtcctagaacgagctggtgcacgtggcttcccaaagatctctcagataatgagaggaaatgcagtcatcagtttgcagaaggctagggattctgggccatagctcagacctgcgcccaccatctccctccaggcagcccttggctggtccctgcgagcccgtggagactgccagtcgctagaaagaggtaagggtttaagggatggttggttggtggggtattaatgtttaattacctggagcacctgcctgaaatcactttttttcaggttggaagcttatggaagatgccaaaaacattaagaagggcccagcgccattctacccactcgaagacgggaccgccggcgagcagctgcacaaagccatgaagcgctacgccctggtgcccggcaccatcgcctttaccgacgcacatatcgaggtggacattacctacgccgagtacttcgagatgagcgttcggctggcagaagctatgaagcgctatgggctgaatacaaaccatcggatcgtggtgtgcagcgagaatagcttgcagttcttcatgcccgtgttgggtgccctgttcatcggtgtggctgtggccccagctaacgacatctacaacgagcgcgagctgctgaacagcatgggcatcagccagcccaccgtcgtattcgtgagcaagaaagggctgcaaaagatcctcaacgtgcaaaagaagctaccgatcatacaaaagatcatcatcatggatagcaagaccgactaccagggcttccaaagcatgtacaccttcgtgacttcccatttgccacccggcttcaacgagtacgacttcgtgcccgagagcttcgaccgggacaaaaccatcgccctgatcatgaacagtagtggcagtaccggattgcccaagggcgtagccctaccgcaccgcaccgcttgtgtccgattcagtcatgcccgcgaccccatcttcggcaaccagatcatccccgacaccgctatcctcagcgtggtgccatttcaccacggcttcggcatgttcaccacgctgggctacttgatctgcggctttcgggtcgtgctcatgtaccgcttcgaggaggagctattcttgcgcagcttgcaagactataagattcaatctgccctgctggtgcccacactatttagcttcttcgctaagagcactctcatcgacaagtacgacctaagcaacttgcacgagatcgccagcggcggggcgccgctcagcaaggaggtaggtgaggccgtggccaaacgcttccacctaccaggcatccgccagggctacggcctgacagaaacaaccagcgccattctgatcacccccgaaggggacgacaagcctggcgcagtaggcaaggtggtgcccttcttcgaggctaaggtggtggacttggacaccggtaagacactgggtgtgaaccagcgcggcgagctgtgcgtccgtggccccatgatcatgagcggctacgttaacaaccccgaggctacaaacgctctcatcgacaaggacggctggctgcacagcggcgacatcgcctactgggacgaggacgagcacttcttcatcgtggaccggctgaagagcctgatcaaatacaagggctaccaggtagccccagccgaactggagagcatcctgctgcaacaccccaacatcttcgacgccggggtcgccggcctgcccgacgacgatgccggcgagctgcccgccgcagtcgtcgtgctggaacacggtaaaaccatgaccgagaaggagatcgtggactatgtggccagccaggttacaaccgccaagaagctgcgcggtggtgttgtgttcgtggacgaggtgcctaaaggactgaccggcaagttggacgcccgcaagatccgcgagattctcattaaggccaagaagggcggcaagatcgccgtgtaattcgaaacgttgagtccatcttgagcatctgacttctggctaaataaaagatctttattttcattagatctgtgtgttggttttttgtgtgcgtcgagatccacggccgcaggaacccctagtgatggagttggccactccctctctgcgcgctcgctcgctcactgaggccgggcgaccaaaggtcgcccgacgcccgggctttgcccgggcggcctcagtgagcgagcgagcgcgcagctgcctgcaggggcgcctgatgcggtattttctccttacgcatctgtgcggtatttcacaccgcatacgtcaaagcaaccatagtacgcgccctgtagcggcgcattaagcgcggcgggtgtggtggttacgcgcagcgtgaccgctacacttgccagcgccctagcgcccgctcctttcgctttcttcccttcctttctcgccacgttcgccggctttccccgtcaagctctaaatcgggggctccctttagggttccgatttagtgctttacggcacctcgaccccaaaaaacttgatttgggtgatggttcacgtagtgggccatcgccctgatagacggtttttcgccctttgacgttggagtccacgttctttaatagtggactcttgttccaaactggaacaacactcaaccctatctcgggctattcttttgatttataagggattttgccgatttcggcctattggttaaaaaatgagctgatttaacaaaaatttaacgcgaattttaacaaaatattaacgtttacaattttatggtgcactctcagtacaatctgctctgatgccgcatagttaagccagccccgacacccgccaacacccgctgacgcgccctgacgggcttgtctgctcccggcatccgcttacagacaagctgtgaccgtctccgggagctgcatgtgtcagaggttttcaccgtcatcaccgaaacgcgcgagacgaaagggcctcgtgatacgcctatttttataggttaatgtcatgataataatggtttcttagacgtcaggtggcacttttcggggaaatgtgcgcggaacccctatttgtttatttttctaaatacattcaaatatgtatccgctcatgagacaataaccctgataaatgcttcaataatattgaaaaaggaagagtatgagtattcaacatttccgtgtcgcccttattcccttttttgcggcattttgccttcctgtttttgctcacccagaaacgctggtgaaagtaaaagatgctgaagatcagttgggtgcacgagtgggttacatcgaactggatctcaacagcggtaagatccttgagagttttcgccccgaagaacgttttccaatgatgagcacttttaaagttctgctatgtggcgcggtattatcccgtattgacgccgggcaagagcaactcggtcgccgcatacactattctcagaatgacttggttgagtactcaccagtcacagaaaagcatcttacggatggcatgacagtaagagaattatgcagtgctgccataaccatgagtgataacactgcggccaacttacttctgacaacgatcggaggaccgaaggagctaaccgcttttttgcacaacatgggggatcatgtaactcgccttgatcgttgggaaccggagctgaatgaagccataccaaacgacgagcgtgacaccacgatgcctgtagcaatggcaacaacgttgcgcaaactattaactggcgaactacttactctagcttcccggcaacaattaatagactggatggaggcggataaagttgcaggaccacttctgcgctcggcccttccggctggctggtttattgctgataaatctggagccggtgagcgtgggtctcgcggtatcattgcagcactggggccagatggtaagccctcccgtatcgtagttatctacacgacggggagtcaggcaactatggatgaacgaaatagacagatcgctgagataggtgcctcactgattaagcattggtaactgtcagaccaagtttactcatatatactttagattgatttaaaacttcatttttaatttaaaaggatctaggtgaagatcctttttgataatctcatgaccaaaatcccttaacgtgagttttcgttccactgagcgtcagaccccgtagaaaagatcaaaggatcttcttgagatcctttttttctgcgcgtaatctgctgcttgcaaacaaaaaaaccaccgctaccagcggtggtttgtttgccggatcaagagctaccaactctttttccgaaggtaactggcttcagcagagcgcagataccaaatactgtccttctagtgtagccgtagttaggccaccacttcaagaactctgtagcaccgcctacatacctcgctctgctaatcctgttaccagtggctgctgccagtggcgataagtcgtgtcttaccgggttggactcaagacgatagttaccggataaggcgcagcggtcgggctgaacggggggttcgtgcacacagcccagcttggagcgaacgacctacaccgaactgagatacctacagcgtgagctatgagaaagcgccacgcttcccgaagggagaaaggcggacaggtatccggtaagcggcagggtcggaacaggagagcgcacgagggagcttccagggggaaacgcctggtatctttatagtcctgtcgggtttcgccacctctgacttgagcgtcgatttttgtgatgctcgtcaggggggcggagcctatggaaaaacgccagcaacgcggcctttttacggttcctggccttttgctggccttttgctc

SEQ ID NO: 8 - DNA, 6929 bp, synthetic construct
  source 1..6929: mol_type = other DNA; note = AAVss-CV-EC-CRE18-IFI27-EC-CRE1b-FVIIIprom-Luc-pA
acatgtcctgcaggcagctgcgcgctcgctcgctcactgaggccgcccgggcaaagcccgggcggcctcagtgagcgagcgagcgcgcagagagggagtggccaactccatcactaggggttcctgcggccggcgcgcctccgggttttccccattcccagctcggctgcaaccgagagacagacggaagaaactgccaatggaaggacgcaaagcgtcaactttgtgttcgcccgccactctcggccaatgtgcgctcgtgtctccggagtcccgccttccgtgtcgggcgcccccttttggcagcacagggacgaaccctacgtctcgccatcttgtgtgtggcacaggtaaatttctggactatctttccacctattctggtcctttttcccacacaaccgatttcttagttcgacagctaagtgcggtggcgataaggccagcgtagcctgttgttctcggatcgcccacgtgagctagatcgctacgtcacgccacgcttgccgagcccggcgccatcttgagtgtggcgttttgatgctccggtaccgagactttttttgaaaaacggaacatctgcctatcgcaaggactactattattctgaaaatcaccttcttcattagaaagtaatatttatcattttattatagaactttgatcttacttcttgtgacttcattctgcgtagagcacactcccatccttgaattaaatgacaaagcattttatattaactgacaatgactgatgccatgggcaaatcctatttctgtaaataactgaattttcttctggactgcgcatgaggggagaaagatgtctgcagtttcggtttcctggaaaatgaaacctatctcatttgttgcctgtgtcaaggggcagtgcttcagtcggggtggagctgcttaaaaggcctgggatcacaccctttgggaacacatccaagcttaagacggtgaggtcagcttcacattctcaggaactctccttctttgggtaagactgggagggtgggcaggagctacccttcccgtggccccggaccttgggtgggctgtgggctcagggagcggaggggaggccttaagcatccactctctgcccggtgtttttgttccgtacgactagtgagctcaccatggctacattctgatgtaaagagatatatcctatacctgggccaaatgtaaacagcctggaaaagtgttaggttaaaaacaaaacaaaataaataaatgaataaatgccaggtggttatgagtgctattgagaaaaatgaagccaagagggatatcagtgatgcaggtgggggtaaagagcttacaacataaatgtggtgttccatatttaaacctcattcaacagggaagattggagctgaaatgtgaaggagttgtgggagtggaactacgtggaaatctgggggaaaggtgttttgggtaaaagaaatagcaagtgttgaggtccaggggcatgagtgtgcttgatattttagggaagagtaaggagaccagtataaccagagtgagatgagactacagaggtcaggagaaagggcatgcagaccatgtgggatgctctaggacctaggccatggtaaagatgtagggttttaccctgatggaggtcagaagccattggaggattctgagaagaggagtgacaggactcgctttatagttttaaattataactataaattatagtttttaaaacaatagttgcctaacctcatgttatatgtaaaactacagttttaaaaactataaattcctcatactggcagcagtgtgaggggcaagggcaaaagcagagagactaacaggttgctggttactcttgctagtgcaagtgaattctagaatcttcgacaacatccagaacttctcttgctgctgccactcaggaagagggttggagtaggctaggaataggagcacaaattaaagctcctgttcactttgacttctccatccctctcctcctttccttaaaggttctgattaaagcagacttatgcccctactgctctcagaagtgaatgggttaagtttagcagcctcccttttgctacttcagttcttcctgtggctgcttcccactgataaaaaggaagcaatcctatcggttactgcttagtgctgagcacatccagtgggtaaagttccttaaaatgctctgcaaagaaattgggacttttcattaaatcagaaattttacttttttcccctcctgggagctaaagatattttagagaagaattaaccttttgcttctccagttgaacatttgtagcaataagtcagcgctgcgatcgcgctagctctagaaagaggtaagggtttaagggatggttggttggtggggtattaatgtttaattacctggagcacctgcctgaaatcactttttttcaggttggaagcttatggaagatgccaaaaacattaagaagggcccagcgccattctacccactcgaagacgggaccgccggcgagcagctgcacaaagccatgaagcgctacgccctggtgcccggcaccatcgcctttaccgacgcacatatcgaggtggacattacctacgccgagtacttcgagatgagcgttcggctggcagaagctatgaagcgctatgggctgaatacaaaccatcggatcgtggtgtgcagcgagaatagcttgcagttcttcatgcccgtgttgggtgccctgttcatcggtgtggctgtggccccagctaacgacatctacaacgagcgcgagctgctgaacagcatgggcatcagccagcccaccgtcgtattcgtgagcaagaaagggctgcaaaagatcctcaacgtgcaaaagaagctaccgatcatacaaaagatcatcatcatggatagcaagaccgactaccagggcttccaaagcatgtacaccttcgtgacttcccatttgccacccggcttcaacgagtacgacttcgtgcccgagagcttcgaccgggacaaaaccatcgccctgatcatgaacagtagtggcagtaccggattgcccaagggcgtagccctaccgcaccgcaccgcttgtgtccgattcagtcatgcccgcgaccccatcttcggcaaccagatcatccccgacaccgctatcctcagcgtggtgccatttcaccacggcttcggcatgttcaccacgctgggctacttgatctgcggctttcgggtcgtgctcatgtaccgcttcgaggaggagctattcttgcgcagcttgcaagactataagattcaatctgccctgctggtgcccacactatttagcttcttcgctaagagcactctcatcgacaagtacgacctaagcaacttgcacgagatcgccagcggcggggcgccgctcagcaaggaggtaggtgaggccgtggccaaacgcttccacctaccaggcatccgccagggctacggcctgacagaaacaaccagcgccattctgatcacccccgaaggggacgacaagcctggcgcagtaggcaaggtggtgcccttcttcgaggctaaggtggtggacttggacaccggtaagacactgggtgtgaaccagcgcggcgagctgtgcgtccgtggccccatgatcatgagcggctacgttaacaaccccgaggctacaaacgctctcatcgacaaggacggctggctgcacagcggcgacatcgcctactgggacgaggacgagcacttcttcatcgtggaccggctgaagagcctgatcaaatacaagggctaccaggtagccccagccgaactggagagcatcctgctgcaacaccccaacatcttcgacgccggggtcgccggcctgcccgacgacgatgccggcgagctgcccgccgcagtcgtcgtgctggaacacggtaaaaccatgaccgagaaggagatcgtggactatgtggccagccaggttacaaccgccaagaagctgcgcggtggtgttgtgttcgtggacgaggtgcctaaaggactgaccggcaagttggacgcccgcaagatccgcgagattctcattaaggccaagaagggcggcaagatcgccgtgtaattcgaaacgttgagtccatcttgagcatctgacttctggctaaataaaagatctttattttcattagatctgtgtgttggttttttgtgtgcgtcgagatccacggccgcaggaacccctagtgatggagttggccactccctctctgcgcgctcgctcgctcactgaggccgggcgaccaaaggtcgcccgacgcccgggctttgcccgggcggcctcagtgagcgagcgagcgcgcagctgcctgcaggggcgcctgatgcggtattttctccttacgcatctgtgcggtatttcacaccgcatacgtcaaagcaaccatagtacgcgccctgtagcggcgcattaagcgcggcgggtgtggtggttacgcgcagcgtgaccgctacacttgccagcgccctagcgcccgctcctttcgctttcttcccttcctttctcgccacgttcgccggctttccccgtcaagctctaaatcgggggctccctttagggttccgatttagtgctttacggcacctcgaccccaaaaaacttgatttgggtgatggttcacgtagtgggccatcgccctgatagacggtttttcgccctttgacgttggagtccacgttctttaatagtggactcttgttccaaactggaacaacactcaaccctatctcgggctattcttttgatttataagggattttgccgatttcggcctattggttaaaaaatgagctgatttaacaaaaatttaacgcgaattttaacaaaatattaacgtttacaattttatggtgcactctcagtacaatctgctctgatgccgcatagttaagccagccccgacacccgccaacacccgctgacgcgccctgacgggcttgtctgctcccggcatccgcttacagacaagctgtgaccgtctccgggagctgcatgtgtcagaggttttcaccgtcatcaccgaaacgcgcgagacgaaagggcctcgtgatacgcctatttttataggttaatgtcatgataataatggtttcttagacgtcaggtggcacttttcggggaaatgtgcgcggaacccctatttgtttatttttctaaatacattcaaatatgtatccgctcatgagacaataaccctgataaatgcttcaataatattgaaaaaggaagagtatgagtattcaacatttccgtgtcgcccttattcccttttttgcggcattttgccttcctgtttttgctcacccagaaacgctggtgaaagtaaaagatgctgaagatcagttgggtgcacgagtgggttacatcgaactggatctcaacagcggtaagatccttgagagttttcgccccgaagaacgttttccaatgatgagcacttttaaagttctgctatgtggcgcggtattatcccgtattgacgccgggcaagagcaactcggtcgccgcatacactattctcagaatgacttggttgagtactcaccagtcacagaaaagcatcttacggatggcatgacagtaagagaattatgcagtgctgccataaccatgagtgataacactgcggccaacttacttctgacaacgatcggaggaccgaaggagctaaccgcttttttgcacaacatgggggatcatgtaactcgccttgatcgttgggaaccggagctgaatgaagccataccaaacgacgagcgtgacaccacgatgcctgtagcaatggcaacaacgttgcgcaaactattaactggcgaactacttactctagcttcccggcaacaattaatagactggatggaggcggataaagttgcaggaccacttctgcgctcggcccttccggctggctggtttattgctgataaatctggagccggtgagcgtgggtctcgcggtatcattgcagcactggggccagatggtaagccctcccgtatcgtagttatctacacgacggggagtcaggcaactatggatgaacgaaatagacagatcgctgagataggtgcctcactgattaagcattggtaactgtcagaccaagtttactcatatatactttagattgatttaaaacttcatttttaatttaaaaggatctaggtgaagatcctttttgataatctcatgaccaaaatcccttaacgtgagttttcgttccactgagcgtcagaccccgtagaaaagatcaaaggatcttcttgagatcctttttttctgcgcgtaatctgctgcttgcaaacaaaaaaaccaccgctaccagcggtggtttgtttgccggatcaagagctaccaactctttttccgaaggtaactggcttcagcagagcgcagataccaaatactgtccttctagtgtagccgtagttaggccaccacttcaagaactctgtagcaccgcctacatacctcgctctgctaatcctgttaccagtggctgctgccagtggcgataagtcgtgtcttaccgggttggactcaagacgatagttaccggataaggcgcagcggtcgggctgaacggggggttcgtgcacacagcccagcttggagcgaacgacctacaccgaactgagatacctacagcgtgagctatgagaaagcgccacgcttcccgaagggagaaaggcggacaggtatccggtaagcggcagggtcggaacaggagagcgcacgagggagcttccagggggaaacgcctggtatctttatagtcctgtcgggtttcgccacctctgacttgagcgtcgatttttgtgatgctcgtcaggggggcggagcctatggaaaaacgccagcaacgcggcctttttacggttcctggccttttgctggccttttgctc

SEQ ID NO: 9 - DNA, 7036 bp, synthetic construct
  source 1..7036: mol_type = other DNA; note = AAVss-CV-EC-CRE18-IFI27-EC-CRE1b-EDN1prom-Luc-pA
acatgtcctgcaggcagctgcgcgctcgctcgctcactgaggccgcccgggcaaagcccgggcggcctcagtgagcgagcgagcgcgcagagagggagtggccaactccatcactaggggttcctgcggccggcgcgcctccgggttttccccattcccagctcggctgcaaccgagagacagacggaagaaactgccaatggaaggacgcaaagcgtcaactttgtgttcgcccgccactctcggccaatgtgcgctcgtgtctccggagtcccgccttccgtgtcgggcgcccccttttggcagcacagggacgaaccctacgtctcgccatcttgtgtgtggcacaggtaaatttctggactatctttccacctattctggtcctttttcccacacaaccgatttcttagttcgacagctaagtgcggtggcgataaggccagcgtagcctgttgttctcggatcgcccacgtgagctagatcgctacgtcacgccacgcttgccgagcccggcgccatcttgagtgtggcgttttgatgctccggtaccgagactttttttgaaaaacggaacatctgcctatcgcaaggactactattattctgaaaatcaccttcttcattagaaagtaatatttatcattttattatagaactttgatcttacttcttgtgacttcattctgcgtagagcacactcccatccttgaattaaatgacaaagcattttatattaactgacaatgactgatgccatgggcaaatcctatttctgtaaataactgaattttcttctggactgcgcatgaggggagaaagatgtctgcagtttcggtttcctggaaaatgaaacctatctcatttgttgcctgtgtcaaggggcagtgcttcagtcggggtggagctgcttaaaaggcctgggatcacaccctttgggaacacatccaagcttaagacggtgaggtcagcttcacattctcaggaactctccttctttgggtaagactgggagggtgggcaggagctacccttcccgtggccccggaccttgggtgggctgtgggctcagggagcggaggggaggccttaagcatccactctctgcccggtgtttttgttccgtacgactagtcttgtgcggggaataaatagaatattctgaggtgcattcctccttcctatgttaggcaacattccttgaccctcctcggcccccaagccaggttgcgtttttttctgccatttagaagggttttcctttttgtcctagtaaaacatcagcccctgtagctcttcatctccccctggtgttcttctcccgccatgtcttaagattggtggcaccgaccaatcttaagatttaagttctgtgtgaaaaacacctttgcttttcaatcagtttatcagcctcctccgcaggggaagtgtggacacacaaaagaacttatcggggcttctcatcagtgatagggaaaagactgggcatgtgcctaaacgagctctgatgttatttttaagctccctttcttgccaatccctcacggatctttctccgatagatgcaaagaacttcagcaaaaaagacccgcaggaaggggcttgaagagaaaagtacgttgatctgccaaaatagtctgacccccagtagtggggcagtgacgagggagagcattcccttgtttgactgagactagaatcggagagacataaaaggaaaatgaagcgagcaacaattaaaaaaaattccccgcacacaacaatacaatctatttaaactgtggctcatacttttcataccaatggtatgactttttttctggagtcccctcttctgattcttgaactccggggctggcagcttgcaaaggggaagcggactccagcactgcacgggcaggtttagcaaaggtctctaatgggtattttctttttcttagccctgcccccgaattgtcagacggcgggcgtctgcctctgaagttagcagtgatttcctttcgggcctggccttatctccggctgcacgttgcctgttggtgactaataacacaataacattgtctggggctggaataaagtcggagctgtttacccccactctaataggggttcaatataaaaagccggcagagagctgtccaagtcagacgcgcctctgcatctgcgccaggcgaacgggtcctgcgcctcctgcagtcccagctctccaccgccgcgtgcgcctgcagacgctccgctcgctgccttctctcctggcaggcgctgccttttctccccgttaaaagggcacttgggctgaaggatcgctttgagatctgaggaacccgcagcgctttgagggacctgaagctgtttttcttcgttttcctttgggttcagtttgaacgggaggtttttgatccctttttttcagaagcgctgcgatcgcgctagctctagaaagaggtaagggtttaagggatggttggttggtggggtattaatgtttaattacctggagcacctgcctgaaatcactttttttcaggttggaagcttatggaagatgccaaaaacattaagaagggcccagcgccattctacccactcgaagacgggaccgccggcgagcagctgcacaaagccatgaagcgctacgccctggtgcccggcaccatcgcctttaccgacgcacatatcgaggtggacattacctacgccgagtacttcgagatgagcgttcggctggcagaagctatgaagcgctatgggctgaatacaaaccatcggatcgtggtgtgcagcgagaatagcttgcagttcttcatgcccgtgttgggtgccctgttcatcggtgtggctgtggccccagctaacgacatctacaacgagcgcgagctgctgaacagcatgggcatcagccagcccaccgtcgtattcgtgagcaagaaagggctgcaaaagatcctcaacgtgcaaaagaagctaccgatcatacaaaagatcatcatcatggatagcaagaccgactaccagggcttccaaagcatgtacaccttcgtgacttcccatttgccacccggcttcaacgagtacgacttcgtgcccgagagcttcgaccgggacaaaaccatcgccctgatcatgaacagtagtggcagtaccggattgcccaagggcgtagccctaccgcaccgcaccgcttgtgtccgattcagtcatgcccgcgaccccatcttcggcaaccagatcatccccgacaccgctatcctcagcgtggtgccatttcaccacggcttcggcatgttcaccacgctgggctacttgatctgcggctttcgggtcgtgctcatgtaccgcttcgaggaggagctattcttgcgcagcttgcaagactataagattcaatctgccctgctggtgcccacactatttagcttcttcgctaagagcactctcatcgacaagtacgacctaagcaacttgcacgagatcgccagcggcggggcgccgctcagcaaggaggtaggtgaggccgtggccaaacgcttccacctaccaggcatccgccagggctacggcctgacagaaacaaccagcgccattctgatcacccccgaaggggacgacaagcctggcgcagtaggcaaggtggtgcccttcttcgaggctaaggtggtggacttggacaccggtaagacactgggtgtgaaccagcgcggcgagctgtgcgtccgtggccccatgatcatgagcggctacgttaacaaccccgaggctacaaacgctctcatcgacaaggacggctggctgcacagcggcgacatcgcctactgggacgaggacgagcacttcttcatcgtggaccggctgaagagcctgatcaaatacaagggctaccaggtagccccagccgaactggagagcatcctgctgcaacaccccaacatcttcgacgccggggtcgccggcctgcccgacgacgatgccggcgagctgcccgccgcagtcgtcgtgctggaacacggtaaaaccatgaccgagaaggagatcgtggactatgtggccagccaggttacaaccgccaagaagctgcgcggtggtgttgtgttcgtggacgaggtgcctaaaggactgaccggcaagttggacgcccgcaagatccgcgagattctcattaaggccaagaagggcggcaagatcgccgtgtaattcgaaacgttgagtccatcttgagcatctgacttctggctaaataaaagatctttattttcattagatctgtgtgttggttttttgtgtgcgtcgagatccacggccgcaggaacccctagtgatggagttggccactccctctctgcgcgctcgctcgctcactgaggccgggcgaccaaaggtcgcccgacgcccgggctttgcccgggcggcctcagtgagcgagcgagcgcgcagctgcctgcaggggcgcctgatgcggtattttctccttacgcatctgtgcggtatttcacaccgcatacgtcaaagcaaccatagtacgcgccctgtagcggcgcattaagcgcggcgggtgtggtggttacgcgcagcgtgaccgctacacttgccagcgccctagcgcccgctcctttcgctttcttcccttcctttctcgccacgttcgccggctttccccgtcaagctctaaatcgggggctccctttagggttccgatttagtgctttacggcacctcgaccccaaaaaacttgatttgggtgatggttcacgtagtgggccatcgccctgatagacggtttttcgccctttgacgttggagtccacgttctttaatagtggactcttgttccaaactggaacaacactcaaccctatctcgggctattcttttgatttataagggattttgccgatttcggcctattggttaaaaaatgagctgatttaacaaaaatttaacgcgaattttaacaaaatattaacgtttacaattttatggtgcactctcagtacaatctgctctgatgccgcatagttaagccagccccgacacccgccaacacccgctgacgcgccctgacgggcttgtctgctcccggcatccgcttacagacaagctgtgaccgtctccgggagctgcatgtgtcagaggttttcaccgtcatcaccgaaacgcgcgagacgaaagggcctcgtgatacgcctatttttataggttaatgtcatgataataatggtttcttagacgtcaggtggcacttttcggggaaatgtgcgcggaacccctatttgtttatttttctaaatacattcaaatatgtatccgctcatgagacaataaccctgataaatgcttcaataatattgaaaaaggaagagtatgagtattcaacatttccgtgtcgcccttattcccttttttgcggcattttgccttcctgtttttgctcacccagaaacgctggtgaaagtaaaagatgctgaagatcagttgggtgcacgagtgggttacatcgaactggatctcaacagcggtaagatccttgagagttttcgccccgaagaacgttttccaatgatgagcacttttaaagttctgctatgtggcgcggtattatcccgtattgacgccgggcaagagcaactcggtcgccgcatacactattctcagaatgacttggttgagtactcaccagtcacagaaaagcatcttacggatggcatgacagtaagagaattatgcagtgctgccataaccatgagtgataacactgcggccaacttacttctgacaacgatcggaggaccgaaggagctaaccgcttttttgcacaacatgggggatcatgtaactcgccttgatcgttgggaaccggagctgaatgaagccataccaaacgacgagcgtgacaccacgatgcctgtagcaatggcaacaacgttgcgcaaactattaactggcgaactacttactctagcttcccggcaacaattaatagactggatggaggcggataaagttgcaggaccacttctgcgctcggcccttccggctggctggtttattgctgataaatctggagccggtgagcgtgggtctcgcggtatcattgcagcactggggccagatggtaagccctcccgtatcgtagttatctacacgacggggagtcaggcaactatggatgaacgaaatagacagatcgctgagataggtgcctcactgattaagcattggtaactgtcagaccaagtttactcatatatactttagattgatttaaaacttcatttttaatttaaaaggatctaggtgaagatcctttttgataatctcatgaccaaaatcccttaacgtgagttttcgttccactgagcgtcagaccccgtagaaaagatcaaaggatcttcttgagatcctttttttctgcgcgtaatctgctgcttgcaaacaaaaaaaccaccgctaccagcggtggtttgtttgccggatcaagagctaccaactctttttccgaaggtaactggcttcagcagagcgcagataccaaatactgtccttctagtgtagccgtagttaggccaccacttcaagaactctgtagcaccgcctacatacctcgctctgctaatcctgttaccagtggctgctgccagtggcgataagtcgtgtcttaccgggttggactcaagacgatagttaccggataaggcgcagcggtcgggctgaacggggggttcgtgcacacagcccagcttggagcgaacgacctacaccgaactgagatacctacagcgtgagctatgagaaagcgccacgcttcccgaagggagaaaggcggacaggtatccggtaagcggcagggtcggaacaggagagcgcacgagggagcttccagggggaaacgcctggtatctttatagtcctgtcgggtttcgccacctctgacttgagcgtcgatttttgtgatgctcgtcaggggggcggagcctatggaaaaacgccagcaacgcggcctttttacggttcctggccttttgctggccttttgctc

SEQ ID NO: 10 - DNA, 5579 bp, synthetic construct
  source 1..5579: mol_type = other DNA; note = AAVss-CV-EC-CRE18-ICAM2-Luc-pA
acatgtcctgcaggcagctgcgcgctcgctcgctcactgaggccgcccgggcaaagcccgggcggcctcagtgagcgagcgagcgcgcagagagggagtggccaactccatcactaggggttcctgcggccggcgcgcctccgggttttccccattcccagctcggctgcaaccgagagacagacggaagaaactgccaatggaaggacgcaaagcgtcaactttgtgttcgcccgccactctcggccaatgtgcgctcgtgtctccggagtcccgccttccgtgtcgggcgcccccttttggcagcacagggacgaaccctacgtctcgccatcttgtgtgtggcacaggtaaatttctggactatctttccacctattctggtcctttttcccacacaaccgatttcttagttcgacagctaagtgcggtggcgataaggccagcgtagcctgttgttctcggatcgcccacgtgagctagatcgctacgtcacgccacgcttgccgagcccggcgccatcttgagtgtggcgttttgatgctccggtacgcggtctagaattcctgcagggcccactagtctcccaggcatgactccaacaatgcatcccatgggatttggggttccccagatctggggcttgtaggcctgactctcccctgtgcacacgtctcatacacgcatgcgtgcacccattgcctgccccgccccttgcacagggagtcagcagggaggactgggttatgccctgcttatcagcagcttcccagcttcctctgcctggattcttagaggcctggggtcctagaacgagctggtgcacgtggcttcccaaagatctctcagataatgagaggaaatgcagtcatcagtttgcagaaggctagggattctgggccatagctcagacctgcgcccaccatctccctccaggcagcccttggctggtccctgcgagcccgtggagactgccagtcgctagaaagaggtaagggtttaagggatggttggttggtggggtattaatgtttaattacctggagcacctgcctgaaatcactttttttcaggttggaagcttatggaagatgccaaaaacattaagaagggcccagcgccattctacccactcgaagacgggaccgccggcgagcagctgcacaaagccatgaagcgctacgccctggtgcccggcaccatcgcctttaccgacgcacatatcgaggtggacattacctacgccgagtacttcgagatgagcgttcggctggcagaagctatgaagcgctatgggctgaatacaaaccatcggatcgtggtgtgcagcgagaatagcttgcagttcttcatgcccgtgttgggtgccctgttcatcggtgtggctgtggccccagctaacgacatctacaacgagcgcgagctgctgaacagcatgggcatcagccagcccaccgtcgtattcgtgagcaagaaagggctgcaaaagatcctcaacgtgcaaaagaagctaccgatcatacaaaagatcatcatcatggatagcaagaccgactaccagggcttccaaagcatgtacaccttcgtgacttcccatttgccacccggcttcaacgagtacgacttcgtgcccgagagcttcgaccgggacaaaaccatcgccctgatcatgaacagtagtggcagtaccggattgcccaagggcgtagccctaccgcaccgcaccgcttgtgtccgattcagtcatgcccgcgaccccatcttcggcaaccagatcatccccgacaccgctatcctcagcgtggtgccatttcaccacggcttcggcatgttcaccacgctgggctacttgatctgcggctttcgggtcgtgctcatgtaccgcttcgaggaggagctattcttgcgcagcttgcaagactataagattcaatctgccctgctggtgcccacactatttagcttcttcgctaagagcactctcatcgacaagtacgacctaagcaacttgcacgagatcgccagcggcggggcgccgctcagcaaggaggtaggtgaggccgtggccaaacgcttccacctaccaggcatccgccagggctacggcctgacagaaacaaccagcgccattctgatcacccccgaaggggacgacaagcctggcgcagtaggcaaggtggtgcccttcttcgaggctaaggtggtggacttggacaccggtaagacactgggtgtgaaccagcgcggcgagctgtgcgtccgtggccccatgatcatgagcggctacgttaacaaccccgaggctacaaacgctctcatcgacaaggacggctggctgcacagcggcgacatcgcctactgggacgaggacgagcacttcttcatcgtggaccggctgaagagcctgatcaaatacaagggctaccaggtagccccagccgaactggagagcatcctgctgcaacaccccaacatcttcgacgccggggtcgccggcctgcccgacgacgatgccggcgagctgcccgccgcagtcgtcgtgctggaacacggtaaaaccatgaccgagaaggagatcgtggactatgtggccagccaggttacaaccgccaagaagctgcgcggtggtgttgtgttcgtggacgaggtgcctaaaggactgaccggcaagttggacgcccgcaagatccgcgagattctcattaaggccaagaagggcggcaagatcgccgtgtaattcgaaacgttgagtccatcttgagcatctgacttctggctaaataaaagatctttattttcattagatctgtgtgttggttttttgtgtgcgtcgagatccacggccgcaggaacccctagtgatggagttggccactccctctctgcgcgctcgctcgctcactgaggccgggcgaccaaaggtcgcccgacgcccgggctttgcccgggcggcctcagtgagcgagcgagcgcgcagctgcctgcaggggcgcctgatgcggtattttctccttacgcatctgtgcggtatttcacaccgcatacgtcaaagcaaccatagtacgcgccctgtagcggcgcattaagcgcggcgggtgtggtggttacgcgcagcgtgaccgctacacttgccagcgccctagcgcccgctcctttcgctttcttcccttcctttctcgccacgttcgccggctttccccgtcaagctctaaatcgggggctccctttagggttccgatttagtgctttacggcacctcgaccccaaaaaacttgatttgggtgatggttcacgtagtgggccatcgccctgatagacggtttttcgccctttgacgttggagtccacgttctttaatagtggactcttgttccaaactggaacaacactcaaccctatctcgggctattcttttgatttataagggattttgccgatttcggcctattggttaaaaaatgagctgatttaacaaaaatttaacgcgaattttaacaaaatattaacgtttacaattttatggtgcactctcagtacaatctgctctgatgccgcatagttaagccagccccgacacccgccaacacccgctgacgcgccctgacgggcttgtctgctcccggcatccgcttacagacaagctgtgaccgtctccgggagctgcatgtgtcagaggttttcaccgtcatcaccgaaacgcgcgagacgaaagggcctcgtgatacgcctatttttataggttaatgtcatgataataatggtttcttagacgtcaggtggcacttttcggggaaatgtgcgcggaacccctatttgtttatttttctaaatacattcaaatatgtatccgctcatgagacaataaccctgataaatgcttcaataatattgaaaaaggaagagtatgagtattcaacatttccgtgtcgcccttattcccttttttgcggcattttgccttcctgtttttgctcacccagaaacgctggtgaaagtaaaagatgctgaagatcagttgggtgcacgagtgggttacatcgaactggatctcaacagcggtaagatccttgagagttttcgccccgaagaacgttttccaatgatgagcacttttaaagttctgctatgtggcgcggtattatcccgtattgacgccgggcaagagcaactcggtcgccgcatacactattctcagaatgacttggttgagtactcaccagtcacagaaaagcatcttacggatggcatgacagtaagagaattatgcagtgctgccataaccatgagtgataacactgcggccaacttacttctgacaacgatcggaggaccgaaggagctaaccgcttttttgcacaacatgggggatcatgtaactcgccttgatcgttgggaaccggagctgaatgaagccataccaaacgacgagcgtgacaccacgatgcctgtagcaatggcaacaacgttgcgcaaactattaactggcgaactacttactctagcttcccggcaacaattaatagactggatggaggcggataaagttgcaggaccacttctgcgctcggcccttccggctggctggtttattgctgataaatctggagccggtgagcgtgggtctcgcggtatcattgcagcactggggccagatggtaagccctcccgtatcgtagttatctacacgacggggagtcaggcaactatggatgaacgaaatagacagatcgctgagataggtgcctcactgattaagcattggtaactgtcagaccaagtttactcatatatactttagattgatttaaaacttcatttttaatttaaaaggatctaggtgaagatcctttttgataatctcatgaccaaaatcccttaacgtgagttttcgttccactgagcgtcagaccccgtagaaaagatcaaaggatcttcttgagatcctttttttctgcgcgtaatctgctgcttgcaaacaaaaaaaccaccgctaccagcggtggtttgtttgccggatcaagagctaccaactctttttccgaaggtaactggcttcagcagagcgcagataccaaatactgtccttctagtgtagccgtagttaggccaccacttcaagaactctgtagcaccgcctacatacctcgctctgctaatcctgttaccagtggctgctgccagtggcgataagtcgtgtcttaccgggttggactcaagacgatagttaccggataaggcgcagcggtcgggctgaacggggggttcgtgcacacagcccagcttggagcgaacgacctacaccgaactgagatacctacagcgtgagctatgagaaagcgccacgcttcccgaagggagaaaggcggacaggtatccggtaagcggcagggtcggaacaggagagcgcacgagggagcttccagggggaaacgcctggtatctttatagtcctgtcgggtttcgccacctctgacttgagcgtcgatttttgtgatgctcgtcaggggggcggagcctatggaaaaacgccagcaacgcggcctttttacggttcctggccttttgctggccttttgctc

SEQ ID NO: 11 - DNA, 5177 bp, synthetic construct
  source 1..5177: mol_type = other DNA; note = AAVss-ICAM2-Luc-pA
acatgtcctgcaggcagctgcgcgctcgctcgctcactgaggccgcccgggcaaagcccgggcggcctcagtgagcgagcgagcgcgcagagagggagtggccaactccatcactaggggttcctgcggccggcgcgccacgcgtggtacgcggtctagaattcctgcagggcccactagtctcccaggcatgactccaacaatgcatcccatgggatttggggttccccagatctggggcttgtaggcctgactctcccctgtgcacacgtctcatacacgcatgcgtgcacccattgcctgccccgccccttgcacagggagtcagcagggaggactgggttatgccctgcttatcagcagcttcccagcttcctctgcctggattcttagaggcctggggtcctagaacgagctggtgcacgtggcttcccaaagatctctcagataatgagaggaaatgcagtcatcagtttgcagaaggctagggattctgggccatagctcagacctgcgcccaccatctccctccaggcagcccttggctggtccctgcgagcccgtggagactgccagtcgctagaaagaggtaagggtttaagggatggttggttggtggggtattaatgtttaattacctggagcacctgcctgaaatcactttttttcaggttggaagcttatggaagatgccaaaaacattaagaagggcccagcgccattctacccactcgaagacgggaccgccggcgagcagctgcacaaagccatgaagcgctacgccctggtgcccggcaccatcgcctttaccgacgcacatatcgaggtggacattacctacgccgagtacttcgagatgagcgttcggctggcagaagctatgaagcgctatgggctgaatacaaaccatcggatcgtggtgtgcagcgagaatagcttgcagttcttcatgcccgtgttgggtgccctgttcatcggtgtggctgtggccccagctaacgacatctacaacgagcgcgagctgctgaacagcatgggcatcagccagcccaccgtcgtattcgtgagcaagaaagggctgcaaaagatcctcaacgtgcaaaagaagctaccgatcatacaaaagatcatcatcatggatagcaagaccgactaccagggcttccaaagcatgtacaccttcgtgacttcccatttgccacccggcttcaacgagtacgacttcgtgcccgagagcttcgaccgggacaaaaccatcgccctgatcatgaacagtagtggcagtaccggattgcccaagggcgtagccctaccgcaccgcaccgcttgtgtccgattcagtcatgcccgcgaccccatcttcggcaaccagatcatccccgacaccgctatcctcagcgtggtgccatttcaccacggcttcggcatgttcaccacgctgggctacttgatctgcggctttcgggtcgtgctcatgtaccgcttcgaggaggagctattcttgcgcagcttgcaagactataagattcaatctgccctgctggtgcccacactatttagcttcttcgctaagagcactctcatcgacaagtacgacctaagcaacttgcacgagatcgccagcggcggggcgccgctcagcaaggaggtaggtgaggccgtggccaaacgcttccacctaccaggcatccgccagggctacggcctgacagaaacaaccagcgccattctgatcacccccgaaggggacgacaagcctggcgcagtaggcaaggtggtgcccttcttcgaggctaaggtggtggacttggacaccggtaagacactgggtgtgaaccagcgcggcgagctgtgcgtccgtggccccatgatcatgagcggctacgttaacaaccccgaggctacaaacgctctcatcgacaaggacggctggctgcacagcggcgacatcgcctactgggacgaggacgagcacttcttcatcgtggaccggctgaagagcctgatcaaatacaagggctaccaggtagccccagccgaactggagagcatcctgctgcaacaccccaacatcttcgacgccggggtcgccggcctgcccgacgacgatgccggcgagctgcccgccgcagtcgtcgtgctggaacacggtaaaaccatgaccgagaaggagatcgtggactatgtggccagccaggttacaaccgccaagaagctgcgcggtggtgttgtgttcgtggacgaggtgcctaaaggactgaccggcaagttggacgcccgcaagatccgcgagattctcattaaggccaagaagggcggcaagatcgccgtgtaattcgaaacgttgagtccatcttgagcatctgacttctggctaaataaaagatctttattttcattagatctgtgtgttggttttttgtgtgcgtcgagatccacggccgcaggaacccctagtgatggagttggccactccctctctgcgcgctcgctcgctcactgaggccgggcgaccaaaggtcgcccgacgcccgggctttgcccgggcggcctcagtgagcgagcgagcgcgcagctgcctgcaggggcgcctgatgcggtattttctccttacgcatctgtgcggtatttcacaccgcatacgtcaaagcaaccatagtacgcgccctgtagcggcgcattaagcgcggcgggtgtggtggttacgcgcagcgtgaccgctacacttgccagcgccctagcgcccgctcctttcgctttcttcccttcctttctcgccacgttcgccggctttccccgtcaagctctaaatcgggggctccctttagggttccgatttagtgctttacggcacctcgaccccaaaaaacttgatttgggtgatggttcacgtagtgggccatcgccctgatagacggtttttcgccctttgacgttggagtccacgttctttaatagtggactcttgttccaaactggaacaacactcaaccctatctcgggctattcttttgatttataagggattttgccgatttcggcctattggttaaaaaatgagctgatttaacaaaaatttaacgcgaattttaacaaaatattaacgtttacaattttatggtgcactctcagtacaatctgctctgatgccgcatagttaagccagccccgacacccgccaacacccgctgacgcgccctgacgggcttgtctgctcccggcatccgcttacagacaagctgtgaccgtctccgggagctgcatgtgtcagaggttttcaccgtcatcaccgaaacgcgcgagacgaaagggcctcgtgatacgcctatttttataggttaatgtcatgataataatggtttcttagacgtcaggtggcacttttcggggaaatgtgcgcggaacccctatttgtttatttttctaaatacattcaaatatgtatccgctcatgagacaataaccctgataaatgcttcaataatattgaaaaaggaagagtatgagtattcaacatttccgtgtcgcccttattcccttttttgcggcattttgccttcctgtttttgctcacccagaaacgctggtgaaagtaaaagatgctgaagatcagttgggtgcacgagtgggttacatcgaactggatctcaacagcggtaagatccttgagagttttcgccccgaagaacgttttccaatgatgagcacttttaaagttctgctatgtggcgcggtattatcccgtattgacgccgggcaagagcaactcggtcgccgcatacactattctcagaatgacttggttgagtactcaccagtcacagaaaagcatcttacggatggcatgacagtaagagaattatgcagtgctgccataaccatgagtgataacactgcggccaacttacttctgacaacgatcggaggaccgaaggagctaaccgcttttttgcacaacatgggggatcatgtaactcgccttgatcgttgggaaccggagctgaatgaagccataccaaacgacgagcgtgacaccacgatgcctgtagcaatggcaacaacgttgcgcaaactattaactggcgaactacttactctagcttcccggcaacaattaatagactggatggaggcggataaagttgcaggaccacttctgcgctcggcccttccggctggctggtttattgctgataaatctggagccggtgagcgtgggtctcgcggtatcattgcagcactggggccagatggtaagccctcccgtatcgtagttatctacacgacggggagtcaggcaactatggatgaacgaaatagacagatcgctgagataggtgcctcactgattaagcattggtaactgtcagaccaagtttactcatatatactttagattgatttaaaacttcatttttaatttaaaaggatctaggtgaagatcctttttgataatctcatgaccaaaatcccttaacgtgagttttcgttccactgagcgtcagaccccgtagaaaagatcaaaggatcttcttgagatcctttttttctgcgcgtaatctgctgcttgcaaacaaaaaaaccaccgctaccagcggtggtttgtttgccggatcaagagctaccaactctttttccgaaggtaactggcttcagcagagcgcagataccaaatactgttcttctagtgtagccgtagttaggccaccacttcaagaactctgtagcaccgcctacatacctcgctctgctaatcctgttaccagtggctgctgccagtggcgataagtcgtgtcttaccgggttggactcaagacgatagttaccggataaggcgcagcggtcgggctgaacggggggttcgtgcacacagcccagcttggagcgaacgacctacaccgaactgagatacctacagcgtgagctatgagaaagcgccacgcttcccgaagggagaaaggcggacaggtatccggtaagcggcagggtcggaacaggagagcgcacgagggagcttccagggggaaacgcctggtatctttatagtcctgtcgggtttcgccacctctgacttgagcgtcgatttttgtgatgctcgtcaggggggcggagcctatggaaaaacgccagcaacgcggcctttttacggttcctggccttttgctggccttttgctc

SEQ ID NO: 12 - DNA, 20 bp, synthetic construct
  source 1..20: mol_type = other DNA; note = luciferase-specific forward primer
cccaccgtcgtattcgtgag

SEQ ID NO: 13 - DNA, 21 bp, synthetic construct
  source 1..21: mol_type = other DNA; note = luciferase-specific reverse primer
tcagggcgatggttttgtccc

SEQ ID NO: 14 - DNA, 5959 bp, synthetic construct
  source 1..5959: mol_type = other DNA; note = AAVss-FVIIIpromoter-Luc-pA
acatgtcctgcaggcagctgcgcgctcgctcgctcactgaggccgcccgggcaaagcccgggcggcctcagtgagcgagcgagcgcgcagagagggagtggccaactccatcactaggggttcctgcggccggcgcgccacgcgtggcgcgcccgtacgactagtgagctcaccatggctacattctgatgtaaagagatatatcctatacctgggccaaatgtaaacagcctggaaaagtgttaggttaaaaacaaaacaaaataaataaatgaataaatgccaggtggttatgagtgctattgagaaaaatgaagccaagagggatatcagtgatgcaggtgggggtaaagagcttacaacataaatgtggtgttccatatttaaacctcattcaacagggaagattggagctgaaatgtgaaggagttgtgggagtggaactacgtggaaatctgggggaaaggtgttttgggtaaaagaaatagcaagtgttgaggtccaggggcatgagtgtgcttgatattttagggaagagtaaggagaccagtataaccagagtgagatgagactacagaggtcaggagaaagggcatgcagaccatgtgggatgctctaggacctaggccatggtaaagatgtagggttttaccctgatggaggtcagaagccattggaggattctgagaagaggagtgacaggactcgctttatagttttaaattataactataaattatagtttttaaaacaatagttgcctaacctcatgttatatgtaaaactacagttttaaaaactataaattcctcatactggcagcagtgtgaggggcaagggcaaaagcagagagactaacaggttgctggttactcttgctagtgcaagtgaattctagaatcttcgacaacatccagaacttctcttgctgctgccactcaggaagagggttggagtaggctaggaataggagcacaaattaaagctcctgttcactttgacttctccatccctctcctcctttccttaaaggttctgattaaagcagacttatgcccctactgctctcagaagtgaatgggttaagtttagcagcctcccttttgctacttcagttcttcctgtggctgcttcccactgataaaaaggaagcaatcctatcggttactgcttagtgctgagcacatccagtgggtaaagttccttaaaatgctctgcaaagaaattgggacttttcattaaatcagaaattttacttttttcccctcctgggagctaaagatattttagagaagaattaaccttttgcttctccagttgaacatttgtagcaataagtcagcgctgcgatcgcgctagctctagaaagaggtaagggtttaagggatggttggttggtggggtattaatgtttaattacctggagcacctgcctgaaatcactttttttcaggttggaagcttatggaagatgccaaaaacattaagaagggcccagcgccattctacccactcgaagacgggaccgccggcgagcagctgcacaaagccatgaagcgctacgccctggtgcccggcaccatcgcctttaccgacgcacatatcgaggtggacattacctacgccgagtacttcgagatgagcgttcggctggcagaagctatgaagcgctatgggctgaatacaaaccatcggatcgtggtgtgcagcgagaatagcttgcagttcttcatgcccgtgttgggtgccctgttcatcggtgtggctgtggccccagctaacgacatctacaacgagcgcgagctgctgaacagcatgggcatcagccagcccaccgtcgtattcgtgagcaagaaagggctgcaaaagatcctcaacgtgcaaaagaagctaccgatcatacaaaagatcatcatcatggatagcaagaccgactaccagggcttccaaagcatgtacaccttcgtgacttcccatttgccacccggcttcaacgagtacgacttcgtgcccgagagcttcgaccgggacaaaaccatcgccctgatcatgaacagtagtggcagtaccggattgcccaagggcgtagccctaccgcaccgcaccgcttgtgtccgattcagtcatgcccgcgaccccatcttcggcaaccagatcatccccgacaccgctatcctcagcgtggtgccatttcaccacggcttcggcatgttcaccacgctgggctacttgatctgcggctttcgggtcgtgctcatgtaccgcttcgaggaggagctattcttgcgcagcttgcaagactataagattcaatctgccctgctggtgcccacactatttagcttcttcgctaagagcactctcatcgacaagtacgacctaagcaacttgcacgagatcgccagcggcggggcgccgctcagcaaggaggtaggtgaggccgtggccaaacgcttccacctaccaggcatccgccagggctacggcctgacagaaacaaccagcgccattctgatcacccccgaaggggacgacaagcctggcgcagtaggcaaggtggtgcccttcttcgaggctaaggtggtggacttggacaccggtaagacactgggtgtgaaccagcgcggcgagctgtgcgtccgtggccccatgatcatgagcggctacgttaacaaccccgaggctacaaacgctctcatcgacaaggacggctggctgcacagcggcgacatcgcctactgggacgaggacgagcacttcttcatcgtggaccggctgaagagcctgatcaaatacaagggctaccaggtagccccagccgaactggagagcatcctgctgcaacaccccaacatcttcgacgccggggtcgccggcctgcccgacgacgatgccggcgagctgcccgccgcagtcgtcgtgctggaacacggtaaaaccatgaccgagaaggagatcgtggactatgtggccagccaggttacaaccgccaagaagctgcgcggtggtgttgtgttcgtggacgaggtgcctaaaggactgaccggcaagttggacgcccgcaagatccgcgagattctcattaaggccaagaagggcggcaagatcgccgtgtaattcgaaacgttgagtccatcttgagcatctgacttctggctaaataaaagatctttattttcattagatctgtgtgttggttttttgtgtgcgtcgagatccacggccgcaggaacccctagtgatggagttggccactccctctctgcgcgctcgctcgctcactgaggccgggcgaccaaaggtcgcccgacgcccgggctttgcccgggcggcctcagtgagcgagcgagcgcgcagctgcctgcaggggcgcctgatgcggtattttctccttacgcatctgtgcggtatttcacaccgcatacgtcaaagcaaccatagtacgcgccctgtagcggcgcattaagcgcggcgggtgtggtggttacgcgcagcgtgaccgctacacttgccagcgccctagcgcccgctcctttcgctttcttcccttcctttctcgccacgttcgccggctttccccgtcaagctctaaatcgggggctccctttagggttccgatttagtgctttacggcacctcgaccccaaaaaacttgatttgggtgatggttcacgtagtgggccatcgccctgatagacggtttttcgccctttgacgttggagtccacgttctttaatagtggactcttgttccaaactggaacaacactcaaccctatctcgggctattcttttgatttataagggattttgccgatttcggcctattggttaaaaaatgagctgatttaacaaaaatttaacgcgaattttaacaaaatattaacgtttacaattttatggtgcactctcagtacaatctgctctgatgccgcatagttaagccagccccgacacccgccaacacccgctgacgcgccctgacgggcttgtctgctcccggcatccgcttacagacaagctgtgaccgtctccgggagctgcatgtgtcagaggttttcaccgtcatcaccgaaacgcgcgagacgaaagggcctcgtgatacgcctatttttataggttaatgtcatgataataatggtttcttagacgtcaggtggcacttttcggggaaatgtgcgcggaacccctatttgtttatttttctaaatacattcaaatatgtatccgctcatgagacaataaccctgataaatgcttcaataatattgaaaaaggaagagtatgagtattcaacatttccgtgtcgcccttattcccttttttgcggcattttgccttcctgtttttgctcacccagaaacgctggtgaaagtaaaagatgctgaagatcagttgggtgcacgagtgggttacatcgaactggatctcaacagcggtaagatccttgagagttttcgccccgaagaacgttttccaatgatgagcacttttaaagttctgctatgtggcgcggtattatcccgtattgacgccgggcaagagcaactcggtcgccgcatacactattctcagaatgacttggttgagtactcaccagtcacagaaaagcatcttacggatggcatgacagtaagagaattatgcagtgctgccataaccatgagtgataacactgcggccaacttacttctgacaacgatcggaggaccgaaggagctaaccgcttttttgcacaacatgggggatcatgtaactcgccttgatcgttgggaaccggagctgaatgaagccataccaaacgacgagcgtgacaccacgatgcctgtagcaatggcaacaacgttgcgcaaactattaactggcgaactacttactctagcttcccggcaacaattaatagactggatggaggcggataaagttgcaggaccacttctgcgctcggcccttccggctggctggtttattgctgataaatctggagccggtgagcgtgggtctcgcggtatcattgcagcactggggccagatggtaagccctcccgtatcgtagttatctacacgacggggagtcaggcaactatggatgaacgaaatagacagatcgctgagataggtgcctcactgattaagcattggtaactgtcagaccaagtttactcatatatactttagattgatttaaaacttcatttttaatttaaaaggatctaggtgaagatcctttttgataatctcatgaccaaaatcccttaacgtgagttttcgttccactgagcgtcagaccccgtagaaaagatcaaaggatcttcttgagatcctttttttctgcgcgtaatctgctgcttgcaaacaaaaaaaccaccgctaccagcggtggtttgtttgccggatcaagagctaccaactctttttccgaaggtaactggcttcagcagagcgcagataccaaatactgtccttctagtgtagccgtagttaggccaccacttcaagaactctgtagcaccgcctacatacctcgctctgctaatcctgttaccagtggctgctgccagtggcgataagtcgtgtcttaccgggttggactcaagacgatagttaccggataaggcgcagcggtcgggctgaacggggggttcgtgcacacagcccagcttggagcgaacgacctacaccgaactgagatacctacagcgtgagctatgagaaagcgccacgcttcccgaagggagaaaggcggacaggtatccggtaagcggcagggtcggaacaggagagcgcacgagggagcttccagggggaaacgcctggtatctttatagtcctgtcgggtttcgccacctctgacttgagcgtcgatttttgtgatgctcgtcaggggggcggagcctatggaaaaacgccagcaacgcggcctttttacggttcctggccttttgctggccttttgctc

SEQ ID NO: 15 - DNA, 6093 bp, synthetic construct
  source 1..6093: mol_type = other DNA; note = AAVss-CV-EC-CRE16- IFI27-EC-CRE1b-ICAM2-Luc-pA
acatgtcctgcaggcagctgcgcgctcgctcgctcactgaggccgcccgggcaaagcccgggcggcctcagtgagcgagcgagcgcgcagagagggagtggccaactccatcactaggggttcctgcggccggcgcgccagacacccaagacattcacagactcagaagtatgtttttattgtgatatggaccatcaaatgccaggaaactcaaagggaaaggctgatactccatccataattcatgccatgggatctgaattcttgcactattatcaatgactcagcaaatgtttgtgtgtgcctgggcggtaaagtgggaaatagtggcttcttataacttcatccaactttgacttaccccagcccctttgattgacagcaggtcagagttgggagaaaaagatctttgaatttgtgtgcaaaatggttaagatgcactaattttgacttgtaagcaagtatttatctagcaaatgctttttggtaccgagactttttttgaaaaacggaacatctgcctatcgcaaggactactattattctgaaaatcaccttcttcattagaaagtaatatttatcattttattatagaactttgatcttacttcttgtgacttcattctgcgtagagcacactcccatccttgaattaaatgacaaagcattttatattaactgacaatgactgatgccatgggcaaatcctatttctgtaaataactgaattttcttctggactgcgcatgaggggagaaagatgtctgcagtttcggtttcctggaaaatgaaacctatctcatttgttgcctgtgtcaaggggcagtgcttcagtcggggtggagctgcttaaaaggcctgggatcacaccctttgggaacacatccaagcttaagacggtgaggtcagcttcacattctcaggaactctccttctttgggtaagactgggagggtgggcaggagctacccttcccgtggccccggaccttgggtgggctgtgggctcagggagcggaggggaggccttaagcatccactctctgcccggtgtttttgttccgtacgcggtctagaattcctgcagggcccactagtctcccaggcatgactccaacaatgcatcccatgggatttggggttccccagatctggggcttgtaggcctgactctcccctgtgcacacgtctcatacacgcatgcgtgcacccattgcctgccccgccccttgcacagggagtcagcagggaggactgggttatgccctgcttatcagcagcttcccagcttcctctgcctggattcttagaggcctggggtcctagaacgagctggtgcacgtggcttcccaaagatctctcagataatgagaggaaatgcagtcatcagtttgcagaaggctagggattctgggccatagctcagacctgcgcccaccatctccctccaggcagcccttggctggtccctgcgagcccgtggagactgccagtcgctagaaagaggtaagggtttaagggatggttggttggtggggtattaatgtttaattacctggagcacctgcctgaaatcactttttttcaggttggaagcttatggaagatgccaaaaacattaagaagggcccagcgccattctacccactcgaagacgggaccgccggcgagcagctgcacaaagccatgaagcgctacgccctggtgcccggcaccatcgcctttaccgacgcacatatcgaggtggacattacctacgccgagtacttcgagatgagcgttcggctggcagaagctatgaagcgctatgggctgaatacaaaccatcggatcgtggtgtgcagcgagaatagcttgcagttcttcatgcccgtgttgggtgccctgttcatcggtgtggctgtggccccagctaacgacatctacaacgagcgcgagctgctgaacagcatgggcatcagccagcccaccgtcgtattcgtgagcaagaaagggctgcaaaagatcctcaacgtgcaaaagaagctaccgatcatacaaaagatcatcatcatggatagcaagaccgactaccagggcttccaaagcatgtacaccttcgtgacttcccatttgccacccggcttcaacgagtacgacttcgtgcccgagagcttcgaccgggacaaaaccatcgccctgatcatgaacagtagtggcagtaccggattgcccaagggcgtagccctaccgcaccgcaccgcttgtgtccgattcagtcatgcccgcgaccccatcttcggcaaccagatcatccccgacaccgctatcctcagcgtggtgccatttcaccacggcttcggcatgttcaccacgctgggctacttgatctgcggctttcgggtcgtgctcatgtaccgcttcgaggaggagctattcttgcgcagcttgcaagactataagattcaatctgccctgctggtgcccacactatttagcttcttcgctaagagcactctcatcgacaagtacgacctaagcaacttgcacgagatcgccagcggcggggcgccgctcagcaaggaggtaggtgaggccgtggccaaacgcttccacctaccaggcatccgccagggctacggcctgacagaaacaaccagcgccattctgatcacccccgaaggggacgacaagcctggcgcagtaggcaaggtggtgcccttcttcgaggctaaggtggtggacttggacaccggtaagacactgggtgtgaaccagcgcggcgagctgtgcgtccgtggccccatgatcatgagcggctacgttaacaaccccgaggctacaaacgctctcatcgacaaggacggctggctgcacagcggcgacatcgcctactgggacgaggacgagcacttcttcatcgtggaccggctgaagagcctgatcaaatacaagggctaccaggtagccccagccgaactggagagcatcctgctgcaacaccccaacatcttcgacgccggggtcgccggcctgcccgacgacgatgccggcgagctgcccgccgcagtcgtcgtgctggaacacggtaaaaccatgaccgagaaggagatcgtggactatgtggccagccaggttacaaccgccaagaagctgcgcggtggtgttgtgttcgtggacgaggtgcctaaaggactgaccggcaagttggacgcccgcaagatccgcgagattctcattaaggccaagaagggcggcaagatcgccgtgtaattcgaaacgttgagtccatcttgagcatctgacttctggctaaataaaagatctttattttcattagatctgtgtgttggttttttgtgtgcgtcgagatccacggccgcaggaacccctagtgatggagttggccactccctctctgcgcgctcgctcgctcactgaggccgggcgaccaaaggtcgcccgacgcccgggctttgcccgggcggcctcagtgagcgagcgagcgcgcagctgcctgcaggggcgcctgatgcggtattttctccttacgcatctgtgcggtatttcacaccgcatacgtcaaagcaaccatagtacgcgccctgtagcggcgcattaagcgcggcgggtgtggtggttacgcgcagcgtgaccgctacacttgccagcgccctagcgcccgctcctttcgctttcttcccttcctttctcgccacgttcgccggctttccccgtcaagctctaaatcgggggctccctttagggttccgatttagtgctttacggcacctcgaccccaaaaaacttgatttgggtgatggttcacgtagtgggccatcgccctgatagacggtttttcgccctttgacgttggagtccacgttctttaatagtggactcttgttccaaactggaacaacactcaaccctatctcgggctattcttttgatttataagggattttgccgatttcggcctattggttaaaaaatgagctgatttaacaaaaatttaacgcgaattttaacaaaatattaacgtttacaattttatggtgcactctcagtacaatctgctctgatgccgcatagttaagccagccccgacacccgccaacacccgctgacgcgccctgacgggcttgtctgctcccggcatccgcttacagacaagctgtgaccgtctccgggagctgcatgtgtcagaggttttcaccgtcatcaccgaaacgcgcgagacgaaagggcctcgtgatacgcctatttttataggttaatgtcatgataataatggtttcttagacgtcaggtggcacttttcggggaaatgtgcgcggaacccctatttgtttatttttctaaatacattcaaatatgtatccgctcatgagacaataaccctgataaatgcttcaataatattgaaaaaggaagagtatgagtattcaacatttccgtgtcgcccttattcccttttttgcggcattttgccttcctgtttttgctcacccagaaacgctggtgaaagtaaaagatgctgaagatcagttgggtgcacgagtgggttacatcgaactggatctcaacagcggtaagatccttgagagttttcgccccgaagaacgttttccaatgatgagcacttttaaagttctgctatgtggcgcggtattatcccgtattgacgccgggcaagagcaactcggtcgccgcatacactattctcagaatgacttggttgagtactcaccagtcacagaaaagcatcttacggatggcatgacagtaagagaattatgcagtgctgccataaccatgagtgataacactgcggccaacttacttctgacaacgatcggaggaccgaaggagctaaccgcttttttgcacaacatgggggatcatgtaactcgccttgatcgttgggaaccggagctgaatgaagccataccaaacgacgagcgtgacaccacgatgcctgtagcaatggcaacaacgttgcgcaaactattaactggcgaactacttactctagcttcccggcaacaattaatagactggatggaggcggataaagttgcaggaccacttctgcgctcggcccttccggctggctggtttattgctgataaatctggagccggtgagcgtgggtctcgcggtatcattgcagcactggggccagatggtaagccctcccgtatcgtagttatctacacgacggggagtcaggcaactatggatgaacgaaatagacagatcgctgagataggtgcctcactgattaagcattggtaactgtcagaccaagtttactcatatatactttagattgatttaaaacttcatttttaatttaaaaggatctaggtgaagatcctttttgataatctcatgaccaaaatcccttaacgtgagttttcgttccactgagcgtcagaccccgtagaaaagatcaaaggatcttcttgagatcctttttttctgcgcgtaatctgctgcttgcaaacaaaaaaaccaccgctaccagcggtggtttgtttgccggatcaagagctaccaactctttttccgaaggtaactggcttcagcagagcgcagataccaaatactgtccttctagtgtagccgtagttaggccaccacttcaagaactctgtagcaccgcctacatacctcgctctgctaatcctgttaccagtggctgctgccagtggcgataagtcgtgtcttaccgggttggactcaagacgatagttaccggataaggcgcagcggtcgggctgaacggggggttcgtgcacacagcccagcttggagcgaacgacctacaccgaactgagatacctacagcgtgagctatgagaaagcgccacgcttcccgaagggagaaaggcggacaggtatccggtaagcggcagggtcggaacaggagagcgcacgagggagcttccagggggaaacgcctggtatctttatagtcctgtcgggtttcgccacctctgacttgagcgtcgatttttgtgatgctcgtcaggggggcggagcctatggaaaaacgccagcaacgcggcctttttacggttcctggccttttgctggccttttgctc

SEQ ID NO: 16 - DNA, 346 bp, Homo sapiens
  source 1..346: mol_type = genomic DNA; note = CV-EC-CRE16
agacacccaagacattcacagactcagaagtatgtttttattgtgatatggaccatcaaatgccaggaaactcaaagggaaaggctgatactccatccataattcatgccatgggatctgaattcttgcactattatcaatgactcagcaaatgtttgtgtgtgcctgggcggtaaagtgggaaatagtggcttcttataacttcatccaactttgacttaccccagcccctttgattgacagcaggtcagagttgggagaaaaagatctttgaatttgtgtgcaaaatggttaagatgcactaattttgacttgtaagcaagtatttatctagcaaatgcttttt

SEQ ID NO: 17 - DNA, 570 bp, Homo sapiens
  source 1..570: mol_type = genomic DNA; note = IFI27-EC-CRE1b
gagactttttttgaaaaacggaacatctgcctatcgcaaggactactattattctgaaaatcaccttcttcattagaaagtaatatttatcattttattatagaactttgatcttacttcttgtgacttcattctgcgtagagcacactcccatccttgaattaaatgacaaagcattttatattaactgacaatgactgatgccatgggcaaatcctatttctgtaaataactgaattttcttctggactgcgcatgaggggagaaagatgtctgcagtttcggtttcctggaaaatgaaacctatctcatttgttgcctgtgtcaaggggcagtgcttcagtcggggtggagctgcttaaaaggcctgggatcacaccctttgggaacacatccaagcttaagacggtgaggtcagcttcacattctcaggaactctccttctttgggtaagactgggagggtgggcaggagctacccttcccgtggccccggaccttgggtgggctgtgggctcagggagcggaggggaggccttaagcatccactctctgcccggtgtttttgttc

SEQ ID NO: 18 - DNA, 399 bp, Homo sapiens
  source 1..399: mol_type = genomic DNA; note = ICAM2 promoter
gtctcccaggcatgactccaacaatgcatcccatgggatttggggttccccagatctggggcttgtaggcctgactctcccctgtgcacacgtctcatacacgcatgcgtgcacccattgcctgccccgccccttgcacagggagtcagcagggaggactgggttatgccctgcttatcagcagcttcccagcttcctctgcctggattcttagaggcctggggtcctagaacgagctggtgcacgtggcttcccaaagatctctcagataatgagaggaaatgcagtcatcagtttgcagaaggctagggattctgggccatagctcagacctgcgcccaccatctccctccaggcagcccttggctggtccctgcgagcccgtggagactgccagtc

SEQ ID NO: 19 - DNA, 1175 bp, Homo sapiens
  source 1..1175: mol_type = genomic DNA; note = FVIII promoter
gagctcaccatggctacattctgatgtaaagagatatatcctatacctgggccaaatgtaaacagcctggaaaagtgttaggttaaaaacaaaacaaaataaataaatgaataaatgccaggtggttatgagtgctattgagaaaaatgaagccaagagggatatcagtgatgcaggtgggggtaaagagcttacaacataaatgtggtgttccatatttaaacctcattcaacagggaagattggagctgaaatgtgaaggagttgtgggagtggaactacgtggaaatctgggggaaaggtgttttgggtaaaagaaatagcaagtgttgaggtccaggggcatgagtgtgcttgatattttagggaagagtaaggagaccagtataaccagagtgagatgagactacagaggtcaggagaaagggcatgcagaccatgtgggatgctctaggacctaggccatggtaaagatgtagggttttaccctgatggaggtcagaagccattggaggattctgagaagaggagtgacaggactcgctttatagttttaaattataactataaattatagtttttaaaacaatagttgcctaacctcatgttatatgtaaaactacagttttaaaaactataaattcctcatactggcagcagtgtgaggggcaagggcaaaagcagagagactaacaggttgctggttactcttgctagtgcaagtgaattctagaatcttcgacaacatccagaacttctcttgctgctgccactcaggaagagggttggagtaggctaggaataggagcacaaattaaagctcctgttcactttgacttctccatccctctcctcctttccttaaaggttctgattaaagcagacttatgcccctactgctctcagaagtgaatgggttaagtttagcagcctcccttttgctacttcagttcttcctgtggctgcttcccactgataaaaaggaagcaatcctatcggttactgcttagtgctgagcacatccagtgggtaaagttccttaaaatgctctgcaaagaaattgggacttttcattaaatcagaaattttacttttttcccctcctgggagctaaagatattttagagaagaattaaccttttgcttctccagttgaacatttgtagcaataagtc

SEQ ID NO: 20 - DNA, 1282 bp, Homo sapiens
  source 1..1282: mol_type = genomic DNA; note = EDN1 promoter
cttgtgcggggaataaatagaatattctgaggtgcattcctccttcctatgttaggcaacattccttgaccctcctcggcccccaagccaggttgcgtttttttctgccatttagaagggttttcctttttgtcctagtaaaacatcagcccctgtagctcttcatctccccctggtgttcttctcccgccatgtcttaagattggtggcaccgaccaatcttaagatttaagttctgtgtgaaaaacacctttgcttttcaatcagtttatcagcctcctccgcaggggaagtgtggacacacaaaagaacttatcggggcttctcatcagtgatagggaaaagactgggcatgtgcctaaacgagctctgatgttatttttaagctccctttcttgccaatccctcacggatctttctccgatagatgcaaagaacttcagcaaaaaagacccgcaggaaggggcttgaagagaaaagtacgttgatctgccaaaatagtctgacccccagtagtggggcagtgacgagggagagcattcccttgtttgactgagactagaatcggagagacataaaaggaaaatgaagcgagcaacaattaaaaaaaattccccgcacacaacaatacaatctatttaaactgtggctcatacttttcataccaatggtatgactttttttctggagtcccctcttctgattcttgaactccggggctggcagcttgcaaaggggaagcggactccagcactgcacgggcaggtttagcaaaggtctctaatgggtattttctttttcttagccctgcccccgaattgtcagacggcgggcgtctgcctctgaagttagcagtgatttcctttcgggcctggccttatctccggctgcacgttgcctgttggtgactaataacacaataacattgtctggggctggaataaagtcggagctgtttacccccactctaataggggttcaatataaaaagccggcagagagctgtccaagtcagacgcgcctctgcatctgcgccaggcgaacgggtcctgcgcctcctgcagtcccagctctccaccgccgcgtgcgcctgcagacgctccgctcgctgccttctctcctggcaggcgctgccttttctccccgttaaaagggcacttgggctgaaggatcgctttgagatctgaggaacccgcagcgctttgagggacctgaagctgtttttcttcgttttcctttgggttcagtttgaacgggaggtttttgatccctttttttcaga

SEQ ID NO: 21 - DNA, 92 bp, synthetic construct
  source 1..92: mol_type = other DNA; note = MVM intron
aagaggtaagggtttaagggatggttggttggtggggtattaatgtttaattacctggagcacctgcctgaaatcactttttttcaggttgg

SEQ ID NO: 22 - DNA, 49 bp, synthetic construct
  source 1..49: mol_type = other DNA; note = syntpA
aataaaagatctttattttcattagatctgtgtgttggttttttgtgtg